European Patent Application EP 4 495 139 A1, published January 22, 2025. Title: 特异性结合GPRC5D和CD3的抗原结合分子及其医药用途. Applicant: 江苏恒瑞医药股份有限公司. The sequence listing filed with the application follows.

SEQUENCE LISTING (227 sequences)

SEQ ID NO: 1 - protein, 118 aa, synthetic construct
  REGION 1..118: note = mAb1
EVQLVESGGGLVKPGGSLKLSCAASGFTFSDYGMHWVRQAPEKGLEWVAFISSGSSTIYYADTVKGRFTISRDNAKNTLFLQMTSLRSEDTAIYYCTRLGPNWYFDVWGTGTTVTVSS

SEQ ID NO: 2 - protein, 113 aa, synthetic construct
  REGION 1..113: note = mAb1
DVVMTQTPLSLSVSLGDQASISCRSSQSLVHSNGNTYLYWYLQKPGQSPKLLIYKVSNRFSGVPDRFSGSGSGTDFTLKISRVEAEDLGVYFCSQSTHVPPLTFGAGTKLELK

SEQ ID NO: 3 - protein, 114 aa, synthetic construct
  REGION 1..114: note = mAb24
QVQLQQSDAELVKPGGSVKISCKVSGYTFTDYPIHWMKQRPEQGLEWMGYVFPRDGSTKYNEKFRVKATWTADKSSSTVYMQLNSLTSDDSAVYFCSRELTAYWGQGTTLRVSS

SEQ ID NO: 4 - protein, 112 aa, synthetic construct
  REGION 1..112: note = mAb24
DVVLTQTPLTLSVTIGQPASISCKSSQSLLHSNGKTYLNWLLQRPGQSPRRLIYLVSKLDSGVPDRFAGSGSGTDFTLKITRVEAEDLGVYYCAQGTHFPRTFGGGSKLEIR

SEQ ID NO: 5 - protein, 118 aa, synthetic construct
  REGION 1..118: note = mAb30
EVQLQQSGPELVKPGGSMKISCKASGYSFTGYTMNWVKQSHGKNPEWIGLINPYNGGTRNNQKFKDKATLTVDKSSSTAYMELLSLTSEDSAVYYCTRWGLRLAMDYWGQGTSVTVSS

SEQ ID NO: 6 - protein, 107 aa, synthetic construct
  REGION 1..107: note = mAb30
DIVMTQSQKFMSTSVGDRVSVTCKASQNVGSNVAWYQQKPGQSPKALIYSASYRYSGVPDRFTGSGSGTDFTLTISNVQSEDLAEYFCHQYNSYPPTFGAGTKLALK

SEQ ID NO: 7 - protein, 121 aa, synthetic construct
  REGION 1..121: note = mAb45
EVKLVESGGGLVQPGDFLSLSCAASGFTFTDYYLSWVRQPPGKALEWLAFIRNRAKGYTTEYSASVKGRFTISRDNSQSILYLQMNVLRAEDSATYYCARMGGKGWHFDVWGTGTTVTVSS

SEQ ID NO: 8 - protein, 112 aa, synthetic construct
  REGION 1..112: note = mAb45
DVLMTQSPLSLPVSLGDQASISCRSSQSIVHSNGNTYLEWYLQKPGQSPKLLIYKVSNRFSGVPDRFFGSGSGTDFTLKINRVEAEDLGVYYCFQGSHVPFTFGGGTKLEIK

SEQ ID NO: 9 - protein, 5 aa, synthetic construct
  REGION 1..5: note = mAb1 HCDR1
DYGMH

SEQ ID NO: 10 - protein, 17 aa, synthetic construct
  REGION 1..17: note = mAb1 HCDR2
FISSGSSTIYYADTVKG

SEQ ID NO: 11 - protein, 9 aa, synthetic construct
  REGION 1..9: note = mAb1 HCDR3
LGPNWYFDV

SEQ ID NO: 12 - protein, 16 aa, synthetic construct
  REGION 1..16: note = mAb1 LCDR1
RSSQSLVHSNGNTYLY

SEQ ID NO: 13 - protein, 7 aa, synthetic construct
  REGION 1..7: note = mAb1 LCDR2
KVSNRFS

SEQ ID NO: 14 - protein, 10 aa, synthetic construct
  REGION 1..10: note = mAb1 LCDR3
SQSTHVPPLT

SEQ ID NO: 15 - protein, 5 aa, synthetic construct
  REGION 1..5: note = mAb24 HCDR1
DYPIH

SEQ ID NO: 16 - protein, 17 aa, synthetic construct
  REGION 1..17: note = mAb24 HCDR2
YVFPRDGSTKYNEKFRV

SEQ ID NO: 17 - protein, 5 aa, synthetic construct
  REGION 1..5: note = mAb24 HCDR3
ELTAY

SEQ ID NO: 18 - protein, 16 aa, synthetic construct
  REGION 1..16: note = mAb24 LCDR1
KSSQSLLHSNGKTYLN

SEQ ID NO: 19 - protein, 7 aa, synthetic construct
  REGION 1..7: note = mAb24 LCDR2
LVSKLDS

SEQ ID NO: 20 - protein, 9 aa, synthetic construct
  REGION 1..9: note = mAb24 LCDR3
AQGTHFPRT

SEQ ID NO: 21 - protein, 5 aa, synthetic construct
  REGION 1..5: note = mAb30 HCDR1
GYTMN

SEQ ID NO: 22 - protein, 17 aa, synthetic construct
  REGION 1..17: note = mAb30 HCDR2
LINPYNGGTRNNQKFKD

SEQ ID NO: 23 - protein, 9 aa, synthetic construct
  REGION 1..9: note = mAb30 HCDR3
WGLRLAMDY

SEQ ID NO: 24 - protein, 11 aa, synthetic construct
  REGION 1..11: note = mAb30 LCDR1
KASQNVGSNVA

SEQ ID NO: 25 - protein, 7 aa, synthetic construct
  REGION 1..7: note = mAb30 LCDR2
SASYRYS

SEQ ID NO: 26 - protein, 9 aa, synthetic construct
  REGION 1..9: note = mAb30 LCDR3
HQYNSYPPT

SEQ ID NO: 27 - protein, 5 aa, synthetic construct
  REGION 1..5: note = mAb45 HCDR1
DYYLS

SEQ ID NO: 28 - protein, 19 aa, synthetic construct
  REGION 1..19: note = mAb45 HCDR2
FIRNRAKGYTTEYSASVKG

SEQ ID NO: 29 - protein, 10 aa, synthetic construct
  REGION 1..10: note = mAb45 HCDR3
MGGKGWHFDV

SEQ ID NO: 30 - protein, 16 aa, synthetic construct
  REGION 1..16: note = mAb45 LCDR1
RSSQSIVHSNGNTYLE

SEQ ID NO: 31 - protein, 7 aa, synthetic construct
  REGION 1..7: note = mAb45 LCDR2
KVSNRFS

SEQ ID NO: 32 - protein, 9 aa, synthetic construct
  REGION 1..9: note = mAb45 LCDR3
FQGSHVPFT

SEQ ID NO: 33 - protein, 118 aa, synthetic construct
  REGION 1..118: note = hu1H1
EVQLVESGGGLVKPGGSLRLSCAASGFTFSDYGMHWVRQAPGKGLEWVAFISSGSSTIYYADTVKGRFTISRDNAKNSLYLQMNSLRAEDTAVYYCTRLGPNWYFDVWGQGTTVTVSS

SEQ ID NO: 34 - protein, 118 aa, synthetic construct
  REGION 1..118: note = hu1H2
EVQLVESGGGLVKPGGSLRLSCAASGFTFSDYGMHWVRQAPGKGLEWVAFISSGSSNIYYADTVKGRFTISRDNAKNSLYLQMNSLRAEDTAVYYCTRLGPNWYFDVWGQGTTVTVSS

SEQ ID NO: 35 - protein, 118 aa, synthetic construct
  REGION 1..118: note = hu1H3
EVQLVESGGGLVKPGGSLRLSCAASGFTFSDYGMHWVRQAPGKGLEWVAFISSGSSTQYYADTVKGRFTISRDNAKNSLYLQMNSLRAEDTAVYYCTRLGPNWYFDVWGQGTTVTVSS

SEQ ID NO: 36 - protein, 113 aa, synthetic construct
  REGION 1..113: note = hu1L1
DIVMTQTPLSLSVTPGQPASISCRSSQSLVHSNGNTYLYWYLQKPGQSPQLLIYKVSNRFSGVPDRFSGSGSGTDFTLKISRVEAEDVGVYYCSQSTHVPPLTFGQGTKLEIK

SEQ ID NO: 37 - protein, 113 aa, synthetic construct
  REGION 1..113: note = hu1L2
DVVMTQTPLSLSVTPGQPASISCRSSQSLVHSNGNTYLYWYLQKPGQSPKLLIYKVSNRFSGVPDRFSGSGSGTDFTLKISRVEAEDVGVYYCSQSTHVPPLTFGQGTKLEIK

SEQ ID NO: 38 - protein, 113 aa, synthetic construct
  REGION 1..113: note = hu1L3
DVVMTQTPLSLSVTPGQPASISCRSSQSLVHSSGNTYLYWYLQKPGQSPKLLIYKVSNRFSGVPDRFSGSGSGTDFTLKISRVEAEDVGVYYCSQSTHVPPLTFGQGTKLEIK

SEQ ID NO: 39 - protein, 113 aa, synthetic construct
  REGION 1..113: note = hu1L4
DVVMTQTPLSLSVTPGQPASISCRSSQSLVHSQGNTYLYWYLQKPGQSPKLLIYKVSNRFSGVPDRFSGSGSGTDFTLKISRVEAEDVGVYYCSQSTHVPPLTFGQGTKLEIK

SEQ ID NO: 40 - protein, 113 aa, synthetic construct
  REGION 1..113: note = hu1L5
DVVMTQTPLSLSVTPGQPASISCRSSQSLVHSTGNTYLYWYLQKPGQSPKLLIYKVSNRFSGVPDRFSGSGSGTDFTLKISRVEAEDVGVYYCSQSTHVPPLTFGQGTKLEIK

SEQ ID NO: 41 - protein, 113 aa, synthetic construct
  REGION 1..113: note = hu1L6
DVVMTQTPLSLSVTPGQPASISCRSSQSLVHSNVNTYLYWYLQKPGQSPKLLIYKVSNRFSGVPDRFSGSGSGTDFTLKISRVEAEDVGVYYCSQSTHVPPLTFGQGTKLEIK

SEQ ID NO: 42 - protein, 114 aa, synthetic construct
  REGION 1..114: note = hu24H1
EVQLVQSGAEVKKPGASVKVSCKASGYTFTDYPIHWVRQAPGQGLEWMGYVFPRDGSTKYNEKFRVRVTMTADTSTSTVYMELSSLRSEDTAVYYCSRELTAYWGQGTTVTVSS

SEQ ID NO: 43 - protein, 114 aa, synthetic construct
  REGION 1..114: note = hu24H2
EVQLVQSGAEVKKPGASVKVSCKASGYTFTDYPIHWVRQAPGQGLEWMGYVFPRDGSTKYNEKFRVRVTWTADKSTSTVYMELSSLRSEDTAVYYCSRELTAYWGQGTTVTVSS

SEQ ID NO: 44 - protein, 114 aa, synthetic construct
  REGION 1..114: note = hu24H3
EVQLVQSGAEVKKPGASVKVSCKVSGYTFTDYPIHWMRQAPGQGLEWMGYVFPRDGSTKYNEKFRVRVTWTADKSTSTVYMELSSLRSEDTAVYYCSRELTAYWGQGTTVTVSS

SEQ ID NO: 45 - protein, 112 aa, synthetic construct
  REGION 1..112: note = hu24L1
DVVMTQSPLSLPVTLGQPASISCKSSQSLLHSNGKTYLNWFQQRPGQSPRRLIYLVSKLDSGVPDRFSGSGSGTDFTLKISRVEAEDVGVYYCAQGTHFPRTFGGGTKVEIK

SEQ ID NO: 46 - protein, 112 aa, synthetic construct
  REGION 1..112: note = hu24L2
DVVLTQSPLSLPVTLGQPASISCKSSQSLLHSNGKTYLNWLLQRPGQSPRRLIYLVSKLDSGVPDRFSGSGSGTDFTLKISRVEAEDVGVYYCAQGTHFPRTFGGGTKVEIK

SEQ ID NO: 47 - protein, 112 aa, synthetic construct
  REGION 1..112: note = hu24L3
DVVLTQSPLSLPVTLGQPASISCKSSQSLLHSNVKTYLNWLLQRPGQSPRRLIYLVSKLDSGVPDRFSGSGSGTDFTLKISRVEAEDVGVYYCAQGTHFPRTFGGGTKVEIK

SEQ ID NO: 48 - protein, 112 aa, synthetic construct
  REGION 1..112: note = hu24L4
DVVLTQSPLSLPVTLGQPASISCKSSQSLLHSNLKTYLNWLLQRPGQSPRRLIYLVSKLDSGVPDRFSGSGSGTDFTLKISRVEAEDVGVYYCAQGTHFPRTFGGGTKVEIK

SEQ ID NO: 49 - protein, 112 aa, synthetic construct
  REGION 1..112: note = hu24L5
DVVLTQSPLSLPVTLGQPASISCKSSQSLLHSSGKTYLNWLLQRPGQSPRRLIYLVSKLDSGVPDRFSGSGSGTDFTLKISRVEAEDVGVYYCAQGTHFPRTFGGGTKVEIK

SEQ ID NO: 50 - protein, 112 aa, synthetic construct
  REGION 1..112: note = hu24L6
DVVLTQSPLSLPVTLGQPASISCKSSQSLLHSTGKTYLNWLLQRPGQSPRRLIYLVSKLDSGVPDRFSGSGSGTDFTLKISRVEAEDVGVYYCAQGTHFPRTFGGGTKVEIK

SEQ ID NO: 51 - protein, 118 aa, synthetic construct
  REGION 1..118: note = hu30H1
EVQLVQSGAEVKKPGASVKVSCKASGYSFTGYTMNWVRQAPGQRLEWMGLINPYNGGTRNNQKFKDRVTITVDKSASTAYMELSSLRSEDTAVYYCTRWGLRLAMDYWGQGTTVTVSS

SEQ ID NO: 52 - protein, 118 aa, synthetic construct
  REGION 1..118: note = hu30H2
EVQLVQSGAEVKKPGASVKVSCKASGYSFTGYTMNWVRQAPGKRPEWMGLINPYNGGTRNNQKFKDRVTITVDKSASTAYMELSSLRSEDTAVYYCTRWGLRLAMDYWGQGTTVTVSS

SEQ ID NO: 53 - protein, 118 aa, synthetic construct
  REGION 1..118: note = hu30H3
EVQLVQSGAEVKKPGASVKVSCKASGYSFTGYTMNWVRQAPGKRPEWMGLINPYNGGTRNNQKFKDRVTLTVDKSASTAYMELSSLRSEDTAVYYCTRWGLRLAMDYWGQGTTVTVSS

SEQ ID NO: 54 - protein, 118 aa, synthetic construct
  REGION 1..118: note = hu30H4
EVQLVQSGAEVKKPGASVKVSCKASGYSFTGYTMNWVRQAPGKRPEWMGLINPYSGGTRNNQKFKDRVTLTVDKSASTAYMELSSLRSEDTAVYYCTRWGLRLAMDYWGQGTTVTVSS

SEQ ID NO: 55 - protein, 118 aa, synthetic construct
  REGION 1..118: note = hu30H5
EVQLVQSGAEVKKPGASVKVSCKASGYSFTGYTMNWVRQAPGKRPEWMGLINPYTGGTRNNQKFKDRVTLTVDKSASTAYMELSSLRSEDTAVYYCTRWGLRLAMDYWGQGTTVTVSS

SEQ ID NO: 56 - protein, 107 aa, synthetic construct
  REGION 1..107: note = hu30L1
DIQMTQSPSSVSASVGDRVTITCKASQNVGSNVAWYQQKPGKAPKALIYSASYRYSGVPSRFSGSGSGTDFTLTISSLQPEDFATYYCHQYNSYPPTFGQGTKLEIK

SEQ ID NO: 57 - protein, 107 aa, synthetic construct
  REGION 1..107: note = hu30L2
DIQMTQSPSSVSASVGDRVTITCKASQNVGSNVAWYQQKPGKSPKALIYSASYRYSGVPSRFSGSGSGTDFTLTISSLQPEDFAEYYCHQYNSYPPTFGQGTKLEIK

SEQ ID NO: 58 - protein, 121 aa, synthetic construct
  REGION 1..121: note = hu45H1
EVQLVESGGGLVQPGGSLRLSCAASGFTFSDYYLSWVRQAPGKGLEWVAFIRNRAKGYTTEYSASVKGRFTISRDNAKNSLYLQMNSLRAEDTAVYYCARMGGKGWHFDVWGQGTTVTVSS

SEQ ID NO: 59 - protein, 121 aa, synthetic construct
  REGION 1..121: note = hu45H2
EVQLVESGGGLVQPGGSLRLSCAASGFTFTDYYLSWVRQAPGKGLEWVAFIRNRAKGYTTEYSASVKGRFTISRDNSKSSLYLQMNSLRAEDTAVYYCARMGGKGWHFDVWGQGTTVTVSS

SEQ ID NO: 60 - protein, 121 aa, synthetic construct
  REGION 1..121: note = hu45H3
EVQLVESGGGLVQPGGSLRLSCAASGFTFTDYYLSWVRQAPGKGLEWVAFIRNRAKGYTTEYSASVKGRFTISRDNSQSILYLQMNSLRAEDTAVYYCARMGGKGWHFDVWGQGTTVTVSS

SEQ ID NO: 61 - protein, 121 aa, synthetic construct
  REGION 1..121: note = hu45H4
EVQLVESGGGLVQPGGSLRLSCAASGFTFTDYYLSWVRQAPGKGLEWVAFIRNRAKGYTTEYSASVKGRFTISRDNAKNSLYLQMNSLRAEDTAVYYCARMGGKGWHFDVWGQGTTVTVSS

SEQ ID NO: 62 - protein, 121 aa, synthetic construct
  REGION 1..121: note = hu45H5
EVQLVESGGGLVQPGGSLRLSCAASGFTFTDYYLSWVRQAPGKGLEWVAFIRNRAKGYTTEYSASVKGRFTISRDNSKNSLYLQMNSLRAEDTAVYYCARMGGKGWHFDVWGQGTTVTVSS

SEQ ID NO: 63 - protein, 121 aa, synthetic construct
  REGION 1..121: note = hu45H6
EVQLVESGGGLVQPGGSLRLSCAASGFTFTDYYLSWVRQAPGKGLEWVAFIRNRAKGYTTEYSASVKGRFTISRDNAKNILYLQMNSLRAEDTAVYYCARMGGKGWHFDVWGQGTTVTVSS

SEQ ID NO: 64 - protein, 121 aa, synthetic construct
  REGION 1..121: note = hu45H7
EVQLVESGGGLVQPGGSLRLSCAASGFTFTDYYLSWVRQAPGKGLEWVAFIRNRAKGYTTEYSASVKGRFTISRDNAQNSLYLQMNSLRAEDTAVYYCARMGGKGWHFDVWGQGTTVTVSS

SEQ ID NO: 65 - protein, 121 aa, synthetic construct
  REGION 1..121: note = hu45H8
EVQLVESGGGLVQPGGSLRLSCAASGFTFTDYYLSWVKQAPGKGLEWVAFIRNRAKGYTTEYSASVKGRFTISRDNSKNSLYLQMNSLRAEDTAVYYCARMGGKGWHFDVWGQGTTVTVSS

SEQ ID NO: 66 - protein, 121 aa, synthetic construct
  REGION 1..121: note = hu45H9
EVQLVESGGGLVQPGGSLRLSCAASGFTFTDYYLSWVKQAPGKGLEWVAFIRNRAKGYTTEYSASVKGRFTISRDNAKNILYLQMNSLRAEDTAVYYCARMGGKGWHFDVWGQGTTVTVSS

SEQ ID NO: 67 - protein, 121 aa, synthetic construct
  REGION 1..121: note = hu45H10
EVQLVESGGGLVQPGGSLRLSCAASGFTFTDYYLSWVKQAPGKGLEWVAFIRNRAKGYTTEYSASVKGRFTISRDNAQNSLYLQMNSLRAEDTAVYYCARMGGKGWHFDVWGQGTTVTVSS

SEQ ID NO: 68 - protein, 121 aa, synthetic construct
  REGION 1..121: note = hu45H11
EVQLVESGGGLVQPGGSLRLSCAASGFTFTDYYLSWVKQAPGKGLEWVGFIRNRAKGYTTEYSASVKGRFTISRDNSQSILYLQMNSLRAEDTAVYYCARMGGKGWHFDVWGQGTTVTVSS

SEQ ID NO: 69 - protein, 112 aa, synthetic construct
  REGION 1..112: note = hu45L1
DIVMTQSPLSLPVTPGEPASISCRSSQSIVHSNGNTYLEWYLQKPGQSPQLLIYKVSNRFSGVPDRFSGSGSGTDFTLKISRVEAEDVGVYYCFQGSHVPFTFGGGTKVEIK

SEQ ID NO: 70 - protein, 112 aa, synthetic construct
  REGION 1..112: note = hu45L2
DVVMTQSPLSLPVTPGEPASISCRSSQSIVHSNGNTYLEWYLQKPGQSPKLLIYKVSNRFSGVPDRFSGSGSGTDFTLKISRVEAEDVGVYYCFQGSHVPFTFGGGTKVEIK

SEQ ID NO: 71 - protein, 112 aa, synthetic construct
  REGION 1..112: note = hu45L3
DVVMTQSPLSLPVTPGEPASISCRSSQSIVHSNGNTYLEWYLQKPGQSPKLLIYKVSNRFSGVPDRFFGSGSGTDFTLKINRVEAEDVGVYYCFQGSHVPFTFGGGTKVEIK

SEQ ID NO: 72 - protein, 112 aa, synthetic construct
  REGION 1..112: note = hu45L4
DVVMTQSPLSLPVTPGEPASISCRSSQSIVHSQGNTYLEWYLQKPGQSPKLLIYKVSNRFSGVPDRFFGSGSGTDFTLKINRVEAEDVGVYYCFQGSHVPFTFGGGTKVEIK

SEQ ID NO: 73 - protein, 112 aa, synthetic construct
  REGION 1..112: note = hu45L5
DVVMTQSPLSLPVTPGEPASISCRSSQSIVHSSGNTYLEWYLQKPGQSPKLLIYKVSNRFSGVPDRFFGSGSGTDFTLKINRVEAEDVGVYYCFQGSHVPFTFGGGTKVEIK

SEQ ID NO: 74 - protein, 112 aa, synthetic construct
  REGION 1..112: note = hu45L6
DVVMTQSPLSLPVTPGEPASISCRSSQSIVHSTGNTYLEWYLQKPGQSPKLLIYKVSNRFSGVPDRFFGSGSGTDFTLKINRVEAEDVGVYYCFQGSHVPFTFGGGTKVEIK

SEQ ID NO: 75 - protein, 112 aa, synthetic construct
  REGION 1..112: note = hu45L7
DVVMTQSPLSLPVTPGEPASISCRSSQSIVHSNRNTYLEWYLQKPGQSPKLLIYKVSNRFSGVPDRFFGSGSGTDFTLKINRVEAEDVGVYYCFQGSHVPFTFGGGTKVEIK

SEQ ID NO: 76 - protein, 5 aa, synthetic construct
  REGION 1..5: note = S107E HCDR1
KYAMN

SEQ ID NO: 77 - protein, 19 aa, synthetic construct
  REGION 1..19: note = S107E HCDR2
RIRSKYNNYATYYADSVKD

SEQ ID NO: 78 - protein, 14 aa, synthetic construct
  REGION 1..14: note = S107E HCDR3
HGNFGNEYISYWAY

SEQ ID NO: 79 - protein, 14 aa, synthetic construct
  REGION 1..14: note = S107E LCDR1
GSSTGAVTSGNYPN

SEQ ID NO: 80 - protein, 7 aa, synthetic construct
  REGION 1..7: note = S107E LCDR2
GTKFLAP

SEQ ID NO: 81 - protein, 9 aa, synthetic construct
  REGION 1..9: note = S107E LCDR3
VLWYSNRWV

SEQ ID NO: 82 - protein, 125 aa, synthetic construct
  REGION 1..125: note = S107E-VH
EVQLVESGGGLVQPGGSLKLSCAASGFTFNKYAMNWVRQAPGKGLEWVARIRSKYNNYATYYADSVKDRFTISRDDSKNTAYLQMNNLKTEDTAVYYCVRHGNFGNEYISYWAYWGQGTLVTVSS

SEQ ID NO: 83 - protein, 109 aa, synthetic construct
  REGION 1..109: note = S107E-VL
QTVVTQEPSLTVSPGGTVTLTCGSSTGAVTSGNYPNWVQQKPGQAPRGLIGGTKFLAPGTPARFSGSLLGGKAALTLSGVQPEDEAEYYCVLWYSNRWVFGGGTKLTVL

SEQ ID NO: 84 - protein, 454 aa, synthetic construct
  REGION 1..454: note = OB(A1B0)-linker1-Hole
EVQLVESGGGLVQPGGSLKLSCAASGFTFNKYAMNWVRQAPGKGLEWVARIRSKYNNYATYYADSVKDRFTISRDDSKNTAYLQMNNLKTEDTAVYYCVRHGNFGNEYISYWAYWGQGTLVTVSSGGGGSSGAPRFLTRPKASVVSVGKDATLSCQIVGNPFPQVSWEKDKQPVTAGVRFRLAQDGDLYRLKILDLQLSDSGQYVCRARNAHGEAFACLGLQVDAEADKTHTCPPCPAPEAAGGPSVFLFPPKPKDTLMISRTPEVTCVVVDVSHEDPEVKFNWYVDGVEVHNAKTKPREEQYNSTYRVVSVLTVLHQDWLNGKEYKCKVSNKALPAPIEKTISKAKGQPREPQVCTLPPSRDELTKNQVSLSCAVKGFYPSDIAVEWESNGQPENNYKTTPPVLDSDGSFFLVSKLTVDKSRWQQGNVFSCSVMHEALHNHYTQKSLSLSPGK

SEQ ID NO: 85 - protein, 212 aa, synthetic construct
  REGION 1..212: note = VL-linker2-Titin(A1B0)
QTVVTQEPSLTVSPGGTVTLTCGSSTGAVTSGNYPNWVQQKPGQAPRGLIGGTKFLAPGTPARFSGSLLGGKAALTLSGVQPEDEAEYYCVLWYSNRWVFGGGTKLTVLGGGGSGIPPKIECLPIDISIDEGKVLTVASAFTGEPTPEVTWSTGGRKIHSQEQGRFHIENTDDSTTLTIKDVQKQDGGLYTLTLRNEFGSDSATVNIHIRSI

SEQ ID NO: 86 - protein, 449 aa, synthetic construct
  REGION 1..449: note = Ob(A0B2)-Hole
EVQLVESGGGLVQPGGSLKLSCAASGFTFNKYAMNWVRQAPGKGLEWVARIRSKYNNYATYYADSVKDRFTISRDDSKNTAYLQMNNLKTEDTAVYYCVRHGNFGNEYISYWAYWGQGTLVTVSSSGAPRFLTCPKASVVSVGKDATLSSQIVGNPFPQVSWEKDKQPVTAGVRFRLAQDGDLYRLKILDLQLSDSGQYVSRARNAHGEAFACLGLQVDAEADKTHTCPPCPAPEAAGGPSVFLFPPKPKDTLMISRTPEVTCVVVDVSHEDPEVKFNWYVDGVEVHNAKTKPREEQYNSTYRVVSVLTVLHQDWLNGKEYKCKVSNKALPAPIEKTISKAKGQPREPQVCTLPPSRDELTKNQVSLSCAVKGFYPSDIAVEWESNGQPENNYKTTPPVLDSDGSFFLVSKLTVDKSRWQQGNVFSCSVMHEALHNHYTQKSLSLSPGK

SEQ ID NO: 87 - protein, 207 aa, synthetic construct
  REGION 1..207: note = VL-Titin(A0B2)
QTVVTQEPSLTVSPGGTVTLTCGSSTGAVTSGNYPNWVQQKPGQAPRGLIGGTKFLAPGTPARFSGSLLGGKAALTLSGVQPEDEAEYYCVLWYSNRWVFGGGTKLTVLGIPPKIECLPIDISIDEGKVLTVASCFTGEPTPEVTWSTGGRKIHSQEQGRFHIENTDDSTTLTIKDVQKQDGGLYTLTLRNEFGSDSATVNIHIRSI

SEQ ID NO: 88 - protein, 454 aa, synthetic construct
  REGION 1..454: note = OB(A1B0)-linker3-Knob
EVQLVESGGGLVQPGGSLKLSCAASGFTFNKYAMNWVRQAPGKGLEWVARIRSKYNNYATYYADSVKDRFTISRDDSKNTAYLQMNNLKTEDTAVYYCVRHGNFGNEYISYWAYWGQGTLVTVSSGGGGSSGAPRFLTRPKASVVSVGKDATLSCQIVGNPFPQVSWEKDKQPVTAGVRFRLAQDGDLYRLKILDLQLSDSGQYVCRARNAHGEAFACLGLQVDAEADKTHTCPPCPAPEAAGGPSVFLFPPKPKDTLMISRTPEVTCVVVDVSHEDPEVKFNWYVDGVEVHNAKTKPREEQYNSTYRVVSVLTVLHQDWLNGKEYKCKVSNKALPAPIEKTISKAKGQPREPQVYTLPPCRDELTKNQVSLWCLVKGFYPSDIAVEWESNGQPENNYKTTPPVLDSDGSFFLYSKLTVDKSRWQQGNVFSCSVMHEALHNHYTQKSLSLSPGK

SEQ ID NO: 89 - protein, 449 aa, synthetic construct
  REGION 1..449: note = Ob(A0B2)-Knob
EVQLVESGGGLVQPGGSLKLSCAASGFTFNKYAMNWVRQAPGKGLEWVARIRSKYNNYATYYADSVKDRFTISRDDSKNTAYLQMNNLKTEDTAVYYCVRHGNFGNEYISYWAYWGQGTLVTVSSSGAPRFLTCPKASVVSVGKDATLSSQIVGNPFPQVSWEKDKQPVTAGVRFRLAQDGDLYRLKILDLQLSDSGQYVSRARNAHGEAFACLGLQVDAEADKTHTCPPCPAPEAAGGPSVFLFPPKPKDTLMISRTPEVTCVVVDVSHEDPEVKFNWYVDGVEVHNAKTKPREEQYNSTYRVVSVLTVLHQDWLNGKEYKCKVSNKALPAPIEKTISKAKGQPREPQVYTLPPCRDELTKNQVSLWCLVKGFYPSDIAVEWESNGQPENNYKTTPPVLDSDGSFFLYSKLTVDKSRWQQGNVFSCSVMHEALHNHYTQKSLSLSPGK

SEQ ID NO: 90 - protein, 5 aa, synthetic construct
  REGION 1..5: note = linker1 linker2
GGGGS

SEQ ID NO: 91 - protein, 103 aa, synthetic construct
  REGION 1..103: note = IgG1(CH1)
ASTKGPSVFPLAPSSKSTSGGTAALGCLVKDYFPEPVTVSWNSGALTSGVHTFPAVLQSSGLYSLSSVVTVPSSSLGTQTYICNVNHKPSNTKVDKKVEPKSC

SEQ ID NO: 92 - protein, 227 aa, synthetic construct
  REGION 1..227: note = IgG1Fc(Knob)
DKTHTCPPCPAPEAAGGPSVFLFPPKPKDTLMISRTPEVTCVVVDVSHEDPEVKFNWYVDGVEVHNAKTKPREEQYNSTYRVVSVLTVLHQDWLNGKEYKCKVSNKALPAPIEKTISKAKGQPREPQVYTLPPCRDELTKNQVSLWCLVKGFYPSDIAVEWESNGQPENNYKTTPPVLDSDGSFFLYSKLTVDKSRWQQGNVFSCSVMHEALHNHYTQKSLSLSPGK

SEQ ID NO: 93 - protein, 227 aa, synthetic construct
  REGION 1..227: note = IgG1Fc(Hole)
DKTHTCPPCPAPEAAGGPSVFLFPPKPKDTLMISRTPEVTCVVVDVSHEDPEVKFNWYVDGVEVHNAKTKPREEQYNSTYRVVSVLTVLHQDWLNGKEYKCKVSNKALPAPIEKTISKAKGQPREPQVCTLPPSRDELTKNQVSLSCAVKGFYPSDIAVEWESNGQPENNYKTTPPVLDSDGSFFLVSKLTVDKSRWQQGNVFSCSVMHEALHNHYTQKSLSLSPGK

SEQ ID NO: 94 - protein, 15 aa, synthetic construct
  REGION 1..15: note = linker5
GGGGSGGGGSGGGGS

SEQ ID NO: 95 - skipped

SEQ ID NO: 96 - protein, 107 aa, synthetic construct [sequence omitted]

SEQ ID NO: 97 - protein, 227 aa, synthetic construct
  REGION 1..227: note = IgG1(AA)Fc
DKTHTCPPCPAPEAAGGPSVFLFPPKPKDTLMISRTPEVTCVVVDVSHEDPEVKFNWYVDGVEVHNAKTKPREEQYNSTYRVVSVLTVLHQDWLNGKEYKCKVSNKALPAPIEKTISKAKGQPREPQVYTLPPSRDELTKNQVSLTCLVKGFYPSDIAVEWESNGQPENNYKTTPPVLDSDGSFFLYSKLTVDKSRWQQGNVFSCSVMHEALHNHYTQKSLSLSPGK

SEQ ID NO: 98 - protein, 700 aa, synthetic construct
  REGION 1..700: note = hu1H2-F11-1
EVQLVESGGGLVKPGGSLRLSCAASGFTFSDYGMHWVRQAPGKGLEWVAFISSGSSNIYYADTVKGRFTISRDNAKNSLYLQMNSLRAEDTAVYYCTRLGPNWYFDVWGQGTTVTVSSASTKGPSVFPLAPSSKSTSGGTAALGCLVKDYFPEPVTVSWNSGALTSGVHTFPAVLQSSGLYSLSSVVTVPSSSLGTQTYICNVNHKPSNTKVDKKVEPKSCEVQLVESGGGLVQPGGSLKLSCAASGFTFNKYAMNWVRQAPGKGLEWVARIRSKYNNYATYYADSVKDRFTISRDDSKNTAYLQMNNLKTEDTAVYYCVRHGNFGNEYISYWAYWGQGTLVTVSSGGGGSGGGGSGGGGSQTVVTQEPSLTVSPGGTVTLTCGSSTGAVTSGNYPNWVQQKPGQAPRGLIGGTKFLAPGTPARFSGSLLGGKAALTLSGVQPEDEAEYYCVLWYSNRWVFGGGTKLTVLGGGDKTHTCPPCPAPEAAGGPSVFLFPPKPKDTLMISRTPEVTCVVVDVSHEDPEVKFNWYVDGVEVHNAKTKPREEQYNSTYRVVSVLTVLHQDWLNGKEYKCKVSNKALPAPIEKTISKAKGQPREPQVYTLPPSRDELTKNQVSLTCLVKGFYPSDIAVEWESNGQPENNYKTTPPVLDSDGSFFLYSKLTVDKSRWQQGNVFSCSVMHEALHNHYTQKSLSLSPGK

SEQ ID NO: 99 - protein, 700 aa, synthetic construct
  REGION 1..700: note = hu1H3-F11-1
EVQLVESGGGLVKPGGSLRLSCAASGFTFSDYGMHWVRQAPGKGLEWVAFISSGSSTQYYADTVKGRFTISRDNAKNSLYLQMNSLRAEDTAVYYCTRLGPNWYFDVWGQGTTVTVSSASTKGPSVFPLAPSSKSTSGGTAALGCLVKDYFPEPVTVSWNSGALTSGVHTFPAVLQSSGLYSLSSVVTVPSSSLGTQTYICNVNHKPSNTKVDKKVEPKSCEVQLVESGGGLVQPGGSLKLSCAASGFTFNKYAMNWVRQAPGKGLEWVARIRSKYNNYATYYADSVKDRFTISRDDSKNTAYLQMNNLKTEDTAVYYCVRHGNFGNEYISYWAYWGQGTLVTVSSGGGGSGGGGSGGGGSQTVVTQEPSLTVSPGGTVTLTCGSSTGAVTSGNYPNWVQQKPGQAPRGLIGGTKFLAPGTPARFSGSLLGGKAALTLSGVQPEDEAEYYCVLWYSNRWVFGGGTKLTVLGGGDKTHTCPPCPAPEAAGGPSVFLFPPKPKDTLMISRTPEVTCVVVDVSHEDPEVKFNWYVDGVEVHNAKTKPREEQYNSTYRVVSVLTVLHQDWLNGKEYKCKVSNKALPAPIEKTISKAKGQPREPQVYTLPPSRDELTKNQVSLTCLVKGFYPSDIAVEWESNGQPENNYKTTPPVLDSDGSFFLYSKLTVDKSRWQQGNVFSCSVMHEALHNHYTQKSLSLSPGK

SEQ ID NO: 100 - protein, 220 aa, synthetic construct
  REGION 1..220: note = hu1L1-CL
DIVMTQTPLSLSVTPGQPASISCRSSQSLVHSNGNTYLYWYLQKPGQSPQLLIYKVSNRFSGVPDRFSGSGSGTDFTLKISRVEAEDVGVYYCSQSTHVPPLTFGQGTKLEIKRTVAAPSVFIFPPSDEQLKSGTASVVCLLNNFYPREAKVQWKVDNALQSGNSQESVTEQDSKDSTYSLSSTLTLSKADYEKHKVYACEVTHQGLSSPVTKSFNRGEC

SEQ ID NO: 101 - protein, 220 aa, synthetic construct
  REGION 1..220: note = hu1L3-CL
DVVMTQTPLSLSVTPGQPASISCRSSQSLVHSSGNTYLYWYLQKPGQSPKLLIYKVSNRFSGVPDRFSGSGSGTDFTLKISRVEAEDVGVYYCSQSTHVPPLTFGQGTKLEIKRTVAAPSVFIFPPSDEQLKSGTASVVCLLNNFYPREAKVQWKVDNALQSGNSQESVTEQDSKDSTYSLSSTLTLSKADYEKHKVYACEVTHQGLSSPVTKSFNRGEC

SEQ ID NO: 102 - protein, 220 aa, synthetic construct
  REGION 1..220: note = hu1L4-CL
DVVMTQTPLSLSVTPGQPASISCRSSQSLVHSQGNTYLYWYLQKPGQSPKLLIYKVSNRFSGVPDRFSGSGSGTDFTLKISRVEAEDVGVYYCSQSTHVPPLTFGQGTKLEIKRTVAAPSVFIFPPSDEQLKSGTASVVCLLNNFYPREAKVQWKVDNALQSGNSQESVTEQDSKDSTYSLSSTLTLSKADYEKHKVYACEVTHQGLSSPVTKSFNRGEC

SEQ ID NO: 103 - protein, 696 aa, synthetic construct
  REGION 1..696: note = hu24H2-F11-1
EVQLVQSGAEVKKPGASVKVSCKASGYTFTDYPIHWVRQAPGQGLEWMGYVFPRDGSTKYNEKFRVRVTWTADKSTSTVYMELSSLRSEDTAVYYCSRELTAYWGQGTTVTVSSASTKGPSVFPLAPSSKSTSGGTAALGCLVKDYFPEPVTVSWNSGALTSGVHTFPAVLQSSGLYSLSSVVTVPSSSLGTQTYICNVNHKPSNTKVDKKVEPKSCEVQLVESGGGLVQPGGSLKLSCAASGFTFNKYAMNWVRQAPGKGLEWVARIRSKYNNYATYYADSVKDRFTISRDDSKNTAYLQMNNLKTEDTAVYYCVRHGNFGNEYISYWAYWGQGTLVTVSSGGGGSGGGGSGGGGSQTVVTQEPSLTVSPGGTVTLTCGSSTGAVTSGNYPNWVQQKPGQAPRGLIGGTKFLAPGTPARFSGSLLGGKAALTLSGVQPEDEAEYYCVLWYSNRWVFGGGTKLTVLGGGDKTHTCPPCPAPEAAGGPSVFLFPPKPKDTLMISRTPEVTCVVVDVSHEDPEVKFNWYVDGVEVHNAKTKPREEQYNSTYRVVSVLTVLHQDWLNGKEYKCKVSNKALPAPIEKTISKAKGQPREPQVYTLPPSRDELTKNQVSLTCLVKGFYPSDIAVEWESNGQPENNYKTTPPVLDSDGSFFLYSKLTVDKSRWQQGNVFSCSVMHEALHNHYTQKSLSLSPGK

SEQ ID NO: 104 - protein, 696 aa, synthetic construct
  REGION 1..696: note = hu24H3-F11-1
EVQLVQSGAEVKKPGASVKVSCKVSGYTFTDYPIHWMRQAPGQGLEWMGYVFPRDGSTKYNEKFRVRVTWTADKSTSTVYMELSSLRSEDTAVYYCSRELTAYWGQGTTVTVSSASTKGPSVFPLAPSSKSTSGGTAALGCLVKDYFPEPVTVSWNSGALTSGVHTFPAVLQSSGLYSLSSVVTVPSSSLGTQTYICNVNHKPSNTKVDKKVEPKSCEVQLVESGGGLVQPGGSLKLSCAASGFTFNKYAMNWVRQAPGKGLEWVARIRSKYNNYATYYADSVKDRFTISRDDSKNTAYLQMNNLKTEDTAVYYCVRHGNFGNEYISYWAYWGQGTLVTVSSGGGGSGGGGSGGGGSQTVVTQEPSLTVSPGGTVTLTCGSSTGAVTSGNYPNWVQQKPGQAPRGLIGGTKFLAPGTPARFSGSLLGGKAALTLSGVQPEDEAEYYCVLWYSNRWVFGGGTKLTVLGGGDKTHTCPPCPAPEAAGGPSVFLFPPKPKDTLMISRTPEVTCVVVDVSHEDPEVKFNWYVDGVEVHNAKTKPREEQYNSTYRVVSVLTVLHQDWLNGKEYKCKVSNKALPAPIEKTISKAKGQPREPQVYTLPPSRDELTKNQVSLTCLVKGFYPSDIAVEWESNGQPENNYKTTPPVLDSDGSFFLYSKLTVDKSRWQQGNVFSCSVMHEALHNHYTQKSLSLSPGK

SEQ ID NO: 105 - protein, 219 aa, synthetic construct
  REGION 1..219: note = hu24L2-CL
DVVLTQSPLSLPVTLGQPASISCKSSQSLLHSNGKTYLNWLLQRPGQSPRRLIYLVSKLDSGVPDRFSGSGSGTDFTLKISRVEAEDVGVYYCAQGTHFPRTFGGGTKVEIKRTVAAPSVFIFPPSDEQLKSGTASVVCLLNNFYPREAKVQWKVDNALQSGNSQESVTEQDSKDSTYSLSSTLTLSKADYEKHKVYACEVTHQGLSSPVTKSFNRGEC

SEQ ID NO: 106 - protein, 219 aa, synthetic construct
  REGION 1..219: note = hu24L5-CL
DVVLTQSPLSLPVTLGQPASISCKSSQSLLHSSGKTYLNWLLQRPGQSPRRLIYLVSKLDSGVPDRFSGSGSGTDFTLKISRVEAEDVGVYYCAQGTHFPRTFGGGTKVEIKRTVAAPSVFIFPPSDEQLKSGTASVVCLLNNFYPREAKVQWKVDNALQSGNSQESVTEQDSKDSTYSLSSTLTLSKADYEKHKVYACEVTHQGLSSPVTKSFNRGEC

SEQ ID NO: 107 - protein, 219 aa, synthetic construct
  REGION 1..219: note = hu24L6-CL
DVVLTQSPLSLPVTLGQPASISCKSSQSLLHSTGKTYLNWLLQRPGQSPRRLIYLVSKLDSGVPDRFSGSGSGTDFTLKISRVEAEDVGVYYCAQGTHFPRTFGGGTKVEIKRTVAAPSVFIFPPSDEQLKSGTASVVCLLNNFYPREAKVQWKVDNALQSGNSQESVTEQDSKDSTYSLSSTLTLSKADYEKHKVYACEVTHQGLSSPVTKSFNRGEC

SEQ ID NO: 108 - protein, 700 aa, synthetic construct
  REGION 1..700: note = hu30H4-F11-1
EVQLVQSGAEVKKPGASVKVSCKASGYSFTGYTMNWVRQAPGKRPEWMGLINPYSGGTRNNQKFKDRVTLTVDKSASTAYMELSSLRSEDTAVYYCTRWGLRLAMDYWGQGTTVTVSSASTKGPSVFPLAPSSKSTSGGTAALGCLVKDYFPEPVTVSWNSGALTSGVHTFPAVLQSSGLYSLSSVVTVPSSSLGTQTYICNVNHKPSNTKVDKKVEPKSCEVQLVESGGGLVQPGGSLKLSCAASGFTFNKYAMNWVRQAPGKGLEWVARIRSKYNNYATYYADSVKDRFTISRDDSKNTAYLQMNNLKTEDTAVYYCVRHGNFGNEYISYWAYWGQGTLVTVSSGGGGSGGGGSGGGGSQTVVTQEPSLTVSPGGTVTLTCGSSTGAVTSGNYPNWVQQKPGQAPRGLIGGTKFLAPGTPARFSGSLLGGKAALTLSGVQPEDEAEYYCVLWYSNRWVFGGGTKLTVLGGGDKTHTCPPCPAPEAAGGPSVFLFPPKPKDTLMISRTPEVTCVVVDVSHEDPEVKFNWYVDGVEVHNAKTKPREEQYNSTYRVVSVLTVLHQDWLNGKEYKCKVSNKALPAPIEKTISKAKGQPREPQVYTLPPSRDELTKNQVSLTCLVKGFYPSDIAVEWESNGQPENNYKTTPPVLDSDGSFFLYSKLTVDKSRWQQGNVFSCSVMHEALHNHYTQKSLSLSPGK

SEQ ID NO: 109 - protein, 700 aa, synthetic construct
  REGION 1..700: note = hu30H5-F11-1
EVQLVQSGAEVKKPGASVKVSCKASGYSFTGYTMNWVRQAPGKRPEWMGLINPYTGGTRNNQKFKDRVTLTVDKSASTAYMELSSLRSEDTAVYYCTRWGLRLAMDYWGQGTTVTVSSASTKGPSVFPLAPSSKSTSGGTAALGCLVKDYFPEPVTVSWNSGALTSGVHTFPAVLQSSGLYSLSSVVTVPSSSLGTQTYICNVNHKPSNTKVDKKVEPKSCEVQLVESGGGLVQPGGSLKLSCAASGFTFNKYAMNWVRQAPGKGLEWVARIRSKYNNYATYYADSVKDRFTISRDDSKNTAYLQMNNLKTEDTAVYYCVRHGNFGNEYISYWAYWGQGTLVTVSSGGGGSGGGGSGGGGSQTVVTQEPSLTVSPGGTVTLTCGSSTGAVTSGNYPNWVQQKPGQAPRGLIGGTKFLAPGTPARFSGSLLGGKAALTLSGVQPEDEAEYYCVLWYSNRWVFGGGTKLTVLGGGDKTHTCPPCPAPEAAGGPSVFLFPPKPKDTLMISRTPEVTCVVVDVSHEDPEVKFNWYVDGVEVHNAKTKPREEQYNSTYRVVSVLTVLHQDWLNGKEYKCKVSNKALPAPIEKTISKAKGQPREPQVYTLPPSRDELTKNQVSLTCLVKGFYPSDIAVEWESNGQPENNYKTTPPVLDSDGSFFLYSKLTVDKSRWQQGNVFSCSVMHEALHNHYTQKSLSLSPGK

SEQ ID NO: 110 - protein, 214 aa, synthetic construct
  REGION 1..214: note = hu30L1-CL
DIQMTQSPSSVSASVGDRVTITCKASQNVGSNVAWYQQKPGKAPKALIYSASYRYSGVPSRFSGSGSGTDFTLTISSLQPEDFATYYCHQYNSYPPTFGQGTKLEIKRTVAAPSVFIFPPSDEQLKSGTASVVCLLNNFYPREAKVQWKVDNALQSGNSQESVTEQDSKDSTYSLSSTLTLSKADYEKHKVYACEVTHQGLSSPVTKSFNRGEC

SEQ ID NO: 111 - protein, 214 aa, synthetic construct
  REGION 1..214: note = hu30L2-CL
DIQMTQSPSSVSASVGDRVTITCKASQNVGSNVAWYQQKPGKSPKALIYSASYRYSGVPSRFSGSGSGTDFTLTISSLQPEDFAEYYCHQYNSYPPTFGQGTKLEIKRTVAAPSVFIFPPSDEQLKSGTASVVCLLNNFYPREAKVQWKVDNALQSGNSQESVTEQDSKDSTYSLSSTLTLSKADYEKHKVYACEVTHQGLSSPVTKSFNRGEC

SEQ ID NO: 112 - protein, 451 aa, synthetic construct
  REGION 1..451: note = hu45H4-CH1-Hole
EVQLVESGGGLVQPGGSLRLSCAASGFTFTDYYLSWVRQAPGKGLEWVAFIRNRAKGYTTEYSASVKGRFTISRDNAKNSLYLQMNSLRAEDTAVYYCARMGGKGWHFDVWGQGTTVTVSSASTKGPSVFPLAPSSKSTSGGTAALGCLVKDYFPEPVTVSWNSGALTSGVHTFPAVLQSSGLYSLSSVVTVPSSSLGTQTYICNVNHKPSNTKVDKKVEPKSCDKTHTCPPCPAPEAAGGPSVFLFPPKPKDTLMISRTPEVTCVVVDVSHEDPEVKFNWYVDGVEVHNAKTKPREEQYNSTYRVVSVLTVLHQDWLNGKEYKCKVSNKALPAPIEKTISKAKGQPREPQVCTLPPSRDELTKNQVSLSCAVKGFYPSDIAVEWESNGQPENNYKTTPPVLDSDGSFFLVSKLTVDKSRWQQGNVFSCSVMHEALHNHYTQKSLSLSPGK

SEQ ID NO: 113 - protein, 451 aa, synthetic construct
  REGION 1..451: note = hu45H5-CH1-Hole
EVQLVESGGGLVQPGGSLRLSCAASGFTFTDYYLSWVRQAPGKGLEWVAFIRNRAKGYTTEYSASVKGRFTISRDNSKNSLYLQMNSLRAEDTAVYYCARMGGKGWHFDVWGQGTTVTVSSASTKGPSVFPLAPSSKSTSGGTAALGCLVKDYFPEPVTVSWNSGALTSGVHTFPAVLQSSGLYSLSSVVTVPSSSLGTQTYICNVNHKPSNTKVDKKVEPKSCDKTHTCPPCPAPEAAGGPSVFLFPPKPKDTLMISRTPEVTCVVVDVSHEDPEVKFNWYVDGVEVHNAKTKPREEQYNSTYRVVSVLTVLHQDWLNGKEYKCKVSNKALPAPIEKTISKAKGQPREPQVCTLPPSRDELTKNQVSLSCAVKGFYPSDIAVEWESNGQPENNYKTTPPVLDSDGSFFLVSKLTVDKSRWQQGNVFSCSVMHEALHNHYTQKSLSLSPGK

SEQ ID NO: 114 - protein, 451 aa, synthetic construct
  REGION 1..451: note = hu45H7-CH1-Hole
EVQLVESGGGLVQPGGSLRLSCAASGFTFTDYYLSWVRQAPGKGLEWVAFIRNRAKGYTTEYSASVKGRFTISRDNAQNSLYLQMNSLRAEDTAVYYCARMGGKGWHFDVWGQGTTVTVSSASTKGPSVFPLAPSSKSTSGGTAALGCLVKDYFPEPVTVSWNSGALTSGVHTFPAVLQSSGLYSLSSVVTVPSSSLGTQTYICNVNHKPSNTKVDKKVEPKSCDKTHTCPPCPAPEAAGGPSVFLFPPKPKDTLMISRTPEVTCVVVDVSHEDPEVKFNWYVDGVEVHNAKTKPREEQYNSTYRVVSVLTVLHQDWLNGKEYKCKVSNKALPAPIEKTISKAKGQPREPQVCTLPPSRDELTKNQVSLSCAVKGFYPSDIAVEWESNGQPENNYKTTPPVLDSDGSFFLVSKLTVDKSRWQQGNVFSCSVMHEALHNHYTQKSLSLSPGK

SEQ ID NO: 115 - protein, 451 aa, synthetic construct
  REGION 1..451: note = hu45H8-CH1-Hole
EVQLVESGGGLVQPGGSLRLSCAASGFTFTDYYLSWVKQAPGKGLEWVAFIRNRAKGYTTEYSASVKGRFTISRDNSKNSLYLQMNSLRAEDTAVYYCARMGGKGWHFDVWGQGTTVTVSSASTKGPSVFPLAPSSKSTSGGTAALGCLVKDYFPEPVTVSWNSGALTSGVHTFPAVLQSSGLYSLSSVVTVPSSSLGTQTYICNVNHKPSNTKVDKKVEPKSCDKTHTCPPCPAPEAAGGPSVFLFPPKPKDTLMISRTPEVTCVVVDVSHEDPEVKFNWYVDGVEVHNAKTKPREEQYNSTYRVVSVLTVLHQDWLNGKEYKCKVSNKALPAPIEKTISKAKGQPREPQVCTLPPSRDELTKNQVSLSCAVKGFYPSDIAVEWESNGQPENNYKTTPPVLDSDGSFFLVSKLTVDKSRWQQGNVFSCSVMHEALHNHYTQKSLSLSPGK

SEQ ID NO: 116 - protein, 451 aa, synthetic construct
  REGION 1..451: note = hu45H10-CH1-Hole
EVQLVESGGGLVQPGGSLRLSCAASGFTFTDYYLSWVKQAPGKGLEWVAFIRNRAKGYTTEYSASVKGRFTISRDNAQNSLYLQMNSLRAEDTAVYYCARMGGKGWHFDVWGQGTTVTVSSASTKGPSVFPLAPSSKSTSGGTAALGCLVKDYFPEPVTVSWNSGALTSGVHTFPAVLQSSGLYSLSSVVTVPSSSLGTQTYICNVNHKPSNTKVDKKVEPKSCDKTHTCPPCPAPEAAGGPSVFLFPPKPKDTLMISRTPEVTCVVVDVSHEDPEVKFNWYVDGVEVHNAKTKPREEQYNSTYRVVSVLTVLHQDWLNGKEYKCKVSNKALPAPIEKTISKAKGQPREPQVCTLPPSRDELTKNQVSLSCAVKGFYPSDIAVEWESNGQPENNYKTTPPVLDSDGSFFLVSKLTVDKSRWQQGNVFSCSVMHEALHNHYTQKSLSLSPGK

SEQ ID NO: 117 - protein, 219 aa, synthetic construct
  REGION 1..219: note = hu45L7-CL
DVVMTQSPLSLPVTPGEPASISCRSSQSIVHSNRNTYLEWYLQKPGQSPKLLIYKVSNRFSGVPDRFFGSGSGTDFTLKINRVEAEDVGVYYCFQGSHVPFTFGGGTKVEIKRTVAAPSVFIFPPSDEQLKSGTASVVCLLNNFYPREAKVQWKVDNALQSGNSQESVTEQDSKDSTYSLSSTLTLSKADYEKHKVYACEVTHQGLSSPVTKSFNRGEC

SEQ ID NO: 118 - protein, 448 aa, synthetic construct
  REGION 1..448: note = hu1H3-CH1-Knob
EVQLVESGGGLVKPGGSLRLSCAASGFTFSDYGMHWVRQAPGKGLEWVAFISSGSSTQYYADTVKGRFTISRDNAKNSLYLQMNSLRAEDTAVYYCTRLGPNWYFDVWGQGTTVTVSSASTKGPSVFPLAPSSKSTSGGTAALGCLVKDYFPEPVTVSWNSGALTSGVHTFPAVLQSSGLYSLSSVVTVPSSSLGTQTYICNVNHKPSNTKVDKKVEPKSCDKTHTCPPCPAPEAAGGPSVFLFPPKPKDTLMISRTPEVTCVVVDVSHEDPEVKFNWYVDGVEVHNAKTKPREEQYNSTYRVVSVLTVLHQDWLNGKEYKCKVSNKALPAPIEKTISKAKGQPREPQVYTLPPCRDELTKNQVSLWCLVKGFYPSDIAVEWESNGQPENNYKTTPPVLDSDGSFFLYSKLTVDKSRWQQGNVFSCSVMHEALHNHYTQKSLSLSPGK

SEQ ID NO: 119 - protein, 448 aa, synthetic construct
  REGION 1..448: note = hu1H3-CH1-Hole
EVQLVESGGGLVKPGGSLRLSCAASGFTFSDYGMHWVRQAPGKGLEWVAFISSGSSTQYYADTVKGRFTISRDNAKNSLYLQMNSLRAEDTAVYYCTRLGPNWYFDVWGQGTTVTVSSASTKGPSVFPLAPSSKSTSGGTAALGCLVKDYFPEPVTVSWNSGALTSGVHTFPAVLQSSGLYSLSSVVTVPSSSLGTQTYICNVNHKPSNTKVDKKVEPKSCDKTHTCPPCPAPEAAGGPSVFLFPPKPKDTLMISRTPEVTCVVVDVSHEDPEVKFNWYVDGVEVHNAKTKPREEQYNSTYRVVSVLTVLHQDWLNGKEYKCKVSNKALPAPIEKTISKAKGQPREPQVCTLPPSRDELTKNQVSLSCAVKGFYPSDIAVEWESNGQPENNYKTTPPVLDSDGSFFLVSKLTVDKSRWQQGNVFSCSVMHEALHNHYTQKSLSLSPGK

SEQ ID NO: 120 - protein, 444 aa, synthetic construct
  REGION 1..444: note = hu24H3-CH1-Knob
EVQLVQSGAEVKKPGASVKVSCKVSGYTFTDYPIHWMRQAPGQGLEWMGYVFPRDGSTKYNEKFRVRVTWTADKSTSTVYMELSSLRSEDTAVYYCSRELTAYWGQGTTVTVSSASTKGPSVFPLAPSSKSTSGGTAALGCLVKDYFPEPVTVSWNSGALTSGVHTFPAVLQSSGLYSLSSVVTVPSSSLGTQTYICNVNHKPSNTKVDKKVEPKSCDKTHTCPPCPAPEAAGGPSVFLFPPKPKDTLMISRTPEVTCVVVDVSHEDPEVKFNWYVDGVEVHNAKTKPREEQYNSTYRVVSVLTVLHQDWLNGKEYKCKVSNKALPAPIEKTISKAKGQPREPQVYTLPPCRDELTKNQVSLWCLVKGFYPSDIAVEWESNGQPENNYKTTPPVLDSDGSFFLYSKLTVDKSRWQQGNVFSCSVMHEALHNHYTQKSLSLSPGK

SEQ ID NO: 121 - protein, 444 aa, synthetic construct
  REGION 1..444: note = hu24H3-CH1-Hole
EVQLVQSGAEVKKPGASVKVSCKVSGYTFTDYPIHWMRQAPGQGLEWMGYVFPRDGSTKYNEKFRVRVTWTADKSTSTVYMELSSLRSEDTAVYYCSRELTAYWGQGTTVTVSSASTKGPSVFPLAPSSKSTSGGTAALGCLVKDYFPEPVTVSWNSGALTSGVHTFPAVLQSSGLYSLSSVVTVPSSSLGTQTYICNVNHKPSNTKVDKKVEPKSCDKTHTCPPCPAPEAAGGPSVFLFPPKPKDTLMISRTPEVTCVVVDVSHEDPEVKFNWYVDGVEVHNAKTKPREEQYNSTYRVVSVLTVLHQDWLNGKEYKCKVSNKALPAPIEKTISKAKGQPREPQVCTLPPSRDELTKNQVSLSCAVKGFYPSDIAVEWESNGQPENNYKTTPPVLDSDGSFFLVSKLTVDKSRWQQGNVFSCSVMHEALHNHYTQKSLSLSPGK

SEQ ID NO: 122 - protein, 448 aa, synthetic construct
  REGION 1..448: note = hu30H5-CH1-Knob
EVQLVQSGAEVKKPGASVKVSCKASGYSFTGYTMNWVRQAPGKRPEWMGLINPYTGGTRNNQKFKDRVTLTVDKSASTAYMELSSLRSEDTAVYYCTRWGLRLAMDYWGQGTTVTVSSASTKGPSVFPLAPSSKSTSGGTAALGCLVKDYFPEPVTVSWNSGALTSGVHTFPAVLQSSGLYSLSSVVTVPSSSLGTQTYICNVNHKPSNTKVDKKVEPKSCDKTHTCPPCPAPEAAGGPSVFLFPPKPKDTLMISRTPEVTCVVVDVSHEDPEVKFNWYVDGVEVHNAKTKPREEQYNSTYRVVSVLTVLHQDWLNGKEYKCKVSNKALPAPIEKTISKAKGQPREPQVYTLPPCRDELTKNQVSLWCLVKGFYPSDIAVEWESNGQPENNYKTTPPVLDSDGSFFLYSKLTVDKSRWQQGNVFSCSVMHEALHNHYTQKSLSLSPGK

SEQ ID NO: 123 - protein, 448 aa, synthetic construct
  REGION 1..448: note = hu30H5-CH1-Hole
EVQLVQSGAEVKKPGASVKVSCKASGYSFTGYTMNWVRQAPGKRPEWMGLINPYTGGTRNNQKFKDRVTLTVDKSASTAYMELSSLRSEDTAVYYCTRWGLRLAMDYWGQGTTVTVSSASTKGPSVFPLAPSSKSTSGGTAALGCLVKDYFPEPVTVSWNSGALTSGVHTFPAVLQSSGLYSLSSVVTVPSSSLGTQTYICNVNHKPSNTKVDKKVEPKSCDKTHTCPPCPAPEAAGGPSVFLFPPKPKDTLMISRTPEVTCVVVDVSHEDPEVKFNWYVDGVEVHNAKTKPREEQYNSTYRVVSVLTVLHQDWLNGKEYKCKVSNKALPAPIEKTISKAKGQPREPQVCTLPPSRDELTKNQVSLSCAVKGFYPSDIAVEWESNGQPENNYKTTPPVLDSDGSFFLVSKLTVDKSRWQQGNVFSCSVMHEALHNHYTQKSLSLSPGK

SEQ ID NO: 124 - protein, 451 aa, synthetic construct
  REGION 1..451: note = hu45H10-CH1-Knob
EVQLVESGGGLVQPGGSLRLSCAASGFTFTDYYLSWVKQAPGKGLEWVAFIRNRAKGYTTEYSASVKGRFTISRDNAQNSLYLQMNSLRAEDTAVYYCARMGGKGWHFDVWGQGTTVTVSSASTKGPSVFPLAPSSKSTSGGTAALGCLVKDYFPEPVTVSWNSGALTSGVHTFPAVLQSSGLYSLSSVVTVPSSSLGTQTYICNVNHKPSNTKVDKKVEPKSCDKTHTCPPCPAPEAAGGPSVFLFPPKPKDTLMISRTPEVTCVVVDVSHEDPEVKFNWYVDGVEVHNAKTKPREEQYNSTYRVVSVLTVLHQDWLNGKEYKCKVSNKALPAPIEKTISKAKGQPREPQVYTLPPCRDELTKNQVSLWCLVKGFYPSDIAVEWESNGQPENNYKTTPPVLDSDGSFFLYSKLTVDKSRWQQGNVFSCSVMHEALHNHYTQKSLSLSPGK

SEQ ID NO: 125 - protein, 445 aa, synthetic construct
  REGION 1..445: note = (anti-GPRC5D)
QVQLVQSGAEVKKPGASVKVSCKASGYSFTGYTMNWVRQAPGQGLEWMGLINPYNSDTNYAQKLQGRVTMTTDTSTSTAYMELRSLRSDDTAVYYCARVALRVALDYWGQGTLVTVSSASTKGPSVFPLAPCSRSTSESTAALGCLVKDYFPEPVTVSWNSGALTSGVHTFPAVLQSSGLYSLSSVVTVPSSSLGTKTYTCNVDHKPSNTKVDKRVESKYGPPCPPCPAPEAAGGPSVFLFPPKPKDTLMISRTPEVTCVVVDVSQEDPEVQFNWYVDGVEVHNAKTKPREEQFNSTYRVVSVLTVLHQDWLNGKEYKCKVSNKGLPSSIEKTISKAKGQPREPQVYTLPPSQEEMTKNQVSLTCLVKGFYPSDIAVEWESNGQPENNYKTTPPVLDSDGSFFLYSRLTVDKSRWQEGNVFSCSVMHEALHNHYTQKSLSLSLGK

SEQ ID NO: 126 - protein, 214 aa, synthetic construct
  REGION 1..214: note = (anti-GPRC5D)
DIQMTQSPSSLSASVGDRVTITCKASQNVATHVGWYQQKPGKAPKRLIYSASYRYSGVPSRFSGSGSGTEFTLTISNLQPEDFATYYCQQYNRYPYTFGQGTKLEIKRTVAAPSVFIFPPSDEQLKSGTASVVCLLNNFYPREAKVQWKVDNALQSGNSQESVTEQDSKDSTYSLSSTLTLSKADYEKHKVYACEVTHQGLSSPVTKSFNRGEC

SEQ ID NO: 127 - protein, 452 aa, synthetic construct
  REGION 1..452: note = (anti-CD3E)
EVQLVESGGGLVQPGGSLRLSCAASGFTFNTYAMNWVRQAPGKGLEWVARIRSKYNNYATYYAASVKGRFTISRDDSKNSLYLQMNSLKTEDTAVYYCARHGNFGNSYVSWFAYWGQGTLVTVSSASTKGPSVFPLAPCSRSTSESTAALGCLVKDYFPEPVTVSWNSGALTSGVHTFPAVLQSSGLYSLSSVVTVPSSSLGTKTYTCNVDHKPSNTKVDKRVESKYGPPCPPCPAPEAAGGPSVFLFPPKPKDTLMISRTPEVTCVVVDVSQEDPEVQFNWYVDGVEVHNAKTKPREEQFNSTYRVVSVLTVLHQDWLNGKEYKCKVSNKGLPSSIEKTISKAKGQPREPQVYTLPPSQEEMTKNQVSLTCLVKGFYPSDIAVEWESNGQPENNYKTTPPVLDSDGSFLLYSKLTVDKSRWQEGNVFSCSVMHEALHNHYTQKSLSLSLGK

SEQ ID NO: 128 - protein, 215 aa, synthetic construct
  REGION 1..215: note = (anti-CD3E)
QTVVTQEPSLTVSPGGTVTLTCRSSTGAVTTSNYANWVQQKPGQAPRGLIGGTNKRAPGTPARFSGSLLGGKAALTLSGVQPEDEAEYYCALWYSNLWVFGGGTKLTVLGQPKAAPSVTLFPPSSEELQANKATLVCLISDFYPGAVTVAWKADSSPVKAGVETTTPSKQSNNKYAASSYLSLTPEQWKSHRSYSCQVTHEGSTVEKTVAPTECS

SEQ ID NO: 129 - protein, 16 aa, synthetic construct
  REGION 1..16: note = hu1L3 LCDR1
RSSQSLVHSSGNTYLY

SEQ ID NO: 130 - protein, 16 aa, synthetic construct
  REGION 1..16: note = hu1L4 LCDR1
RSSQSLVHSQGNTYLY

SEQ ID NO: 131 - protein, 16 aa, synthetic construct
  REGION 1..16: note = hu1L5 LCDR1
RSSQSLVHSTGNTYLY

SEQ ID NO: 132 - protein, 16 aa, synthetic construct
  REGION 1..16: note = hu1L6 LCDR1
RSSQSLVHSNVNTYLY

SEQ ID NO: 133 - protein, 17 aa, synthetic construct
  REGION 1..17: note = hu1H2 HCDR2
FISSGSSNIYYADTVKG

SEQ ID NO: 134 - protein, 17 aa, synthetic construct
  REGION 1..17: note = hu1H2 HCDR2
FISSGSSTQYYADTVKG

SEQ ID NO: 135 - protein, 16 aa, synthetic construct
  REGION 1..16: note = hu24L3 LCDR1
KSSQSLLHSNVKTYLN

SEQ ID NO: 136 - protein, 16 aa, synthetic construct
  REGION 1..16: note = hu24L4 LCDR1
KSSQSLLHSNLKTYLN

SEQ ID NO: 137 - protein, 16 aa, synthetic construct
  REGION 1..16: note = hu24L5 LCDR1
KSSQSLLHSSGKTYLN

SEQ ID NO: 138 - protein, 16 aa, synthetic construct
  REGION 1..16: note = hu24L6 LCDR1
KSSQSLLHSTGKTYLN

SEQ ID NO: 139 - protein, 17 aa, synthetic construct
  REGION 1..17: note = hu30H4 HCDR2
LINPYSGGTRNNQKFKD

SEQ ID NO: 140 - protein, 17 aa, synthetic construct
  REGION 1..17: note = hu30H5 HCDR2
LINPYTGGTRNNQKFKD

SEQ ID NO: 141 - protein, 16 aa, synthetic construct
  REGION 1..16: note = hu45L4 LCDR1
RSSQSIVHSQGNTYLE

SEQ ID NO: 142 - protein, 16 aa, synthetic construct
  REGION 1..16: note = hu45L5 LCDR1
RSSQSIVHSSGNTYLE

SEQ ID NO: 143 - protein, 16 aa, synthetic construct
  REGION 1..16: note = hu45L6 LCDR1
RSSQSIVHSTGNTYLE

SEQ ID NO: 144 - protein, 16 aa, synthetic construct
  REGION 1..16: note = hu45L7 LCDR1
RSSQSIVHSNRNTYLE

SEQ ID NO: 145 - protein, 98 aa, synthetic construct
  REGION 1..98: note = Titin T.0
GIPPKIEALPSDISIDEGKVLTVACAFTGEPTPEVTWSCGGRKIHSQEQGRFHIENTDDLTTLIIMDVQKQDGGLYTLSLGNEFGSDSATVNIHIRSI

SEQ ID NO: 146 - protein, 98 aa, synthetic construct
  REGION 1..98: note = Titin T.1
GIPPKIECLPSDISIDEGKVLTVASAFTGEPTPEVTWSTGGRKIHSQEQGRFHIENTDDLTTLIIMDVQKQDGGLYTLSLGNEFGSDSATVNIHIRSI

SEQ ID NO: 147 - protein, 98 aa, synthetic construct
  REGION 1..98: note = Titin T.2
GIPPKIEALPSDISIDEGKCLTVASAFTGEPTPEVTWSTGGRKIHSQEQGRFHIENTDDLTTLIIMDVQKQDGGLYTLSLGNEFGSDSATVNIHIRSI

SEQ ID NO: 148 - protein, 98 aa, synthetic construct
  REGION 1..98: note = Titin T.3
GIPPKIEALPSDISIDEGKVLTVASCFTGEPTPEVTWSTGGRKIHSQEQGRFHIENTDDLTTLIIMDVQKQDGGLYTLSLGNEFGSDSATVNIHIRSI

SEQ ID NO: 149 - protein, 98 aa, synthetic construct
  REGION 1..98: note = Titin T.4
GIPPKIEALPSDISIDEGKVLCVASAFTGEPTPEVTWSTGGRKIHSQEQGRFHIENTDDLTTLIIMDVQKQDGGLYTLSLGNEFGSDSATVNIHIRSI

SEQ ID NO: 150 - protein, 103 aa, synthetic construct
  REGION 1..103: note = Titin T.5
KAGIRGIPPKIECLPSDISIDEGKVLTVASAFTGEPTPEVTWSTGGRKIHSQEQGRFHIENTDDLTTLIIMDVQKQDGGLYTLSLGNEFGSDSATVNIHIRSI

SEQ ID NO: 151 - protein, 103 aa, synthetic construct
  REGION 1..103: note = Titin T.6
KAGIRGIPPKIEALPSDISIDEGKVLTVACAFTGEPTPEVTWSCGGRKIHSQEQGRFHIENTDDLTTLIIMDVQKQDGGLYTLSLGNEFGSDSATVNIHIRSI

SEQ ID NO: 152 - protein, 98 aa, synthetic construct
  REGION 1..98: note = Titin T.7
GIPPKIECLPSDISIDEGKVLTVASAFTGEPTPEVTWSTGGRKIHSQEQGRFHIENTDDLTTLIISDVQKQDGGLYSLSLGNEFGSDSATVNIHIRSI

SEQ ID NO: 153 - protein, 98 aa, synthetic construct
  REGION 1..98: note = Titin T.8
GIPPKIECLPSDISIDEGKVLTVASAFTGEPTPEVTWSTGGRKIHSQEQGRFHIENTDDLTTLIIKDVQRQDGGLYTLTLRNEFGSDSATVNIHIRSI

SEQ ID NO: 154 - protein, 98 aa, synthetic construct
  REGION 1..98: note = Titin T.9
GIWPKIECLPIDLSIDEGKVLMVASAFTGEPTPEVTWSTGGRKIHSQEQGRFHIENTDDLTTLIIMDVQKQDGGLYTLSLGMEFGSDSATVNIHIRSI

SEQ ID NO: 155 - protein, 98 aa, synthetic construct
  REGION 1..98: note = Titin T.10
GIPPKIECLPIDISIDEGKVLTVASAFTGEPTPEVTWSTGGRKIHSQEQGRFHIENTDDLTTLIIKDVQKQDGGLYTLTLRNEFGSDSATVNIHIRSI

SEQ ID NO: 156 - protein, 98 aa, synthetic construct
  REGION 1..98: note = Titin T.11
GIPPKIECLPSDISIDEGKVLTVASAFTGEPTPEVTWSTSGKKISSEEGGRFHIESTEDLTTLIIMDVQKQDGGVYTLSLGNDLGSDSATVNIHIRSI

SEQ ID NO: 157 - protein, 98 aa, synthetic construct
  REGION 1..98: note = Titin T.12
GIPPKIECLPSDISIDEGKVLTVASAFTGEPTPEVTWSTGGRKIHSEEGGRFHIESTEDLTTLIIMDVQKQDGGVYTLSLGNEFGSDSATVNIHIRSI

SEQ ID NO: 158 - protein, 98 aa, synthetic construct
  REGION 1..98: note = Titin T.13
GIPPKIECLPSDISIDEGKVLTVASAFTGEPTPEVTWSTGGRKIHSQEQGRFHIESTEDLTTLIIMDVQKQDGGVYTLSLGNEFGSDSATVNIHIRSI

SEQ ID NO: 159 - protein, 98 aa, synthetic construct
  REGION 1..98: note = Titin T.14
GIPPKIECLPSDISIDEGKVLTVASAFTGEPTPEVTWSTGGRKIHSQEQGRFHIESTEDLTTLIISDVQKQDGGLYSLSLGNEFGSDSATVNIHIRSI

SEQ ID NO: 160 - protein, 103 aa, synthetic construct
  REGION 1..103: note = Titin T.15
KAGIRGIPPKIECLPSDISIDEGKVLTVASAFTGEPTPEVTWSTGGRKIHSQEQGRFHIESTEDLTTLIISDVQKQDGGLYSLSLGNEFGSDSATVNIHIRSI

SEQ ID NO: 161 - protein, 98 aa, synthetic construct
  REGION 1..98: note = Titin T.16
GIPPKIECLPIDISIDEGKVLTVASAFTGEPTPEVTWSTGGRKIHSQEQGRFHIENTDDSTTLTIKDVQKQDGGLYTLTLRNEFGSDSATVNIHIRSI

SEQ ID NO: 162 - protein, 98 aa, synthetic construct
  REGION 1..98: note = Titin T.17
GIPPKIECLPIDISIDEGKCLTVASAFTGEPTPEVTWSTGGRKIHSQEQGRFHIENTDDSTTLTIKDVQKQDGGLYTLTLRNEFGSDSATVNIHIRSI

SEQ ID NO: 163 - protein, 98 aa, synthetic construct
  REGION 1..98: note = Titin T.18
GIPPKIECLPIDISIDEGKVLTVASCFTGEPTPEVTWSTGGRKIHSQEQGRFHIENTDDSTTLTIKDVQKQDGGLYTLTLRNEFGSDSATVNIHIRSI

SEQ ID NO: 164 - protein, 97 aa, synthetic construct
  REGION 1..97: note = Obscurin O.0
SGAPRFLTRPKAFVVSVGKDATLSCQIVGNPTPQVSWEKDQQPVAAGARFRLAQDGDLYRLTILDLALGDSGQYVCRARNAIGEAFAAVGLQVDAEA

SEQ ID NO: 165 - protein, 98 aa, synthetic construct
  REGION 1..98: note = Obscurin OL.0
QGSPPCFLRFPRPVRVVSGAEAELKCVVLGEPPPVVVWEKGGQQLAASERLSFPADGAEHGLLLTAALPTDAGVYVCRARNAAGEAYAAAAVTVLEPP

SEQ ID NO: 166 - protein, 97 aa, synthetic construct
  REGION 1..97: note = Obscurin O.1
SGAPRFLTRPKAFVVSVGKDATLSCQIVGNPTPQVSWEKDQQPVAAGARFRLAQDGDLYRLTILDLALGDSGQYVCRARNAIGEAFACVGLQVDAEA

SEQ ID NO: 167 - protein, 97 aa, synthetic construct
  REGION 1..97: note = Obscurin O.2
SGCPRFLTRPKAFVVSVGKDATLSCQIVGNPTPQVSWEKDQQPVAAGARFRLAQDGDLYRLTILDLALGDSGQYVCRARNAIGEAFAAVGLQVDAEA

SEQ ID NO: 168 - protein, 97 aa, synthetic construct
  REGION 1..97: note = Obscurin O.3
SGAPRFLTCPKAFVVSVGKDATLSCQIVGNPTPQVSWEKDQQPVAAGARFRLAQDGDLYRLTILDLALGDSGQYVCRARNAIGEAFAAVGLQVDAEA

SEQ ID NO: 169 - protein, 97 aa, synthetic construct
  REGION 1..97: note = Obscurin O.4
SGAPRFLTRPKAFVVSVGKDATLSSQIVGNPTPQVSWEKDQQPVAAGARFRLAQDGDLYRLTILDLALGDSGQYVSRARNAIGEAFACVGLQVDAEA

SEQ ID NO: 170 - protein, 97 aa, synthetic construct
  REGION 1..97: note = Obscurin O.5
SGCPRFLTRPKAFVVSVGKDATLSSQIVGNPTPQVSWEKDQQPVAAGARFRLAQDGDLYRLTILDLALGDSGQYVSRARNAIGEAFAAVGLQVDAEA

SEQ ID NO: 171 - protein, 97 aa, synthetic construct
  REGION 1..97: note = Obscurin O.6
SGAPRFLTCPKAFVVSVGKDATLSSQIVGNPTPQVSWEKDQQPVAAGARFRLAQDGDLYRLTILDLALGDSGQYVSRARNAIGEAFAAVGLQVDAEA

SEQ ID NO: 172 - protein, 97 aa, synthetic construct
  REGION 1..97: note = Obscurin O.7
SGAPRFKTRPKAFVVSVGKDATLSSQIVGNPTPQVSWEKDQQPVAAGARFRLAQDGDLYRLKILDLALGDSGQYVSRARNAIGEAFACVGLQVDAEA

SEQ ID NO: 173 - protein, 97 aa, synthetic construct
  REGION 1..97: note = Obscurin O.8
SGAPRFKTRPKAFVVSVGKDATLSSQIVGNPTPQVSWEKDQQPVAAGARFRLAQDGDLYRLHILDLALGDSGQYVSRARNAIGEAFACVGLQVDAEA

SEQ ID NO: 174 - protein, 97 aa, synthetic construct
  REGION 1..97: note = Obscurin O.9
SGAPRFLTRPLAFVVSVGKDATLSSQIVGNPTPQVSWEKDQQPVAAGARFRLAQDGDLYRLKILDLALGDSGQYVSRARNAIGEAFACVGLQVDAEA

SEQ ID NO: 175 - protein, 97 aa, synthetic construct
  REGION 1..97: note = Obscurin O.10
SGAPRFLTRPLAFVVSVGKDATLSSQIVGNPTPQVSWEKDQQPVAAGARFRLAQDGDLYRLHILDLALGDSGQYVSRARNAIGEAFACVGLQVDAEA

SEQ ID NO: 176 - protein, 102 aa, synthetic construct
  REGION 1..102: note = Obscurin O.11
DQPQFSGAPRFLTRPKAFVVSVGKDATLSSQIVGNPTPQVSWEKDQQPVAAGARFRLAQDGDLYRLTILDLALGDSGQYVSRARNAIGEAFACVGLQVDAEA

SEQ ID NO: 177 - protein, 102 aa, synthetic construct
  REGION 1..102: note = Obscurin O.12
DQPQFSGAPRFKTRPKAFVVSVGKDATLSSQIVGNPTPQVSWEKDQQPVAAGARFRLAQDGDLYRLKILDLALGDSGQYVSRARNAIGEAFACVGLQVDAEA

SEQ ID NO: 178 - protein, 102 aa, synthetic construct
  REGION 1..102: note = Obscurin O.13
DQPQFSGAPRFKTRPKAFVVSVGKDATLSSQIVGNPTPQVSWEKDQQPVAAGARFRLAQDGDLYRLHILDLALGDSGQYVSRARNAIGEAFACVGLQVDAEA

SEQ ID NO: 179 - protein, 102 aa, synthetic construct
  REGION 1..102: note = Obscurin O.14
DQPQFSGAPRFRTRPKAFVVSVGKDATLSSQIVGNPTPQVSWEKDQQPVAAGARFRLAQDGDLYRLKILDLALGDSGQYVSRARNAIGEAFACVGLQVDAEA

SEQ ID NO: 180 - protein, 102 aa, synthetic construct
  REGION 1..102: note = Obscurin O.15
DQPQFSGAPRFRTRPKAFVVSVGKDATLSSQIVGNPTPQVSWEKDQQPVAAGARFRLAQDGDLYRLHILDLALGDSGQYVSRARNAIGEAFACVGLQVDAEA

SEQ ID NO: 181 - protein, 102 aa, synthetic construct
  REGION 1..102: note = Obscurin O.16
DQPQFSGAPRFLTRPKAFVVSVGKDATLSCQIVGNPTPQVSWEKDQQPVAAGARFRLAQDGDLYRLTILDLALGDSGQYVCRARNAIGEAFAAVGLQVDAEA

SEQ ID NO: 182 - protein, 98 aa, synthetic construct
  REGION 1..98: note = Obscurin OL.1
QGSPPEFLRFPRPVRVVSGAEAELKCVVLGEPPPVVVWEKGGQQLAASERLSFPADGAEHGLLLTAALPTDAGCYVCRARNAAGEAYAAAAVTVLEPP

SEQ ID NO: 183 - protein, 98 aa, synthetic construct
  REGION 1..98: note = Obscurin OL.2
QGSPPEFLRFPRPVRVVSGAEAELKCVVLGEPPPVVVWEKGGQQLAASERLSFPADGAEHGLLLTAALPTDAGVYVCRARNAACEAYAAAAVTVLEPP

SEQ ID NO: 184 - protein, 98 aa, synthetic construct
  REGION 1..98: note = Obscurin OL.3
QGSPPEFLRFPRPVRVVSGAEAELKCVVLGEPPPVVVWEKGGQQLAASERLSFPADGAEHGLLLTAALPTDAGVYVCRARNAAGECYAAAAVTVLEPP

SEQ ID NO: 185 - protein, 98 aa, synthetic construct
  REGION 1..98: note = Obscurin OL.4
QGSPPEFLRFPRPVRVVSGAEAELKSVVLGEPPPVVVWEKGGQQLAASERLSFPADGAEHGLLLTAALPTDAGCYVSRARNAAGEAYAAAAVTVLEPP

SEQ ID NO: 186 - protein, 98 aa, synthetic construct
  REGION 1..98: note = Obscurin OL.5
QGSPPEFLRFPRPVRVVSGAEAELKSVVLGEPPPVVVWEKGGQQLAASERLSFPADGAEHGLLLTAALPTDAGVYVSRARNAACEAYAAAAVTVLEPP

SEQ ID NO: 187 - protein, 98 aa, synthetic construct
  REGION 1..98: note = Obscurin OL.6
QGSPPEFLRFPRPVRVVSGAEAELKSVVLGEPPPVVVWEKGGQQLAASERLSFPADGAEHGLLLTAALPTDAGVYVSRARNAAGECYAAAAVTVLEPP

SEQ ID NO: 188 - protein, 97 aa, synthetic construct
  REGION 1..97: note = Obscurin O.17
SGAPRFLTRPKSYTVSVGKDASLSSQIVGNPTPQVSWEKDQQPVAAGARFRLAQDGDLYRLKILDLALGDSGQYVSRARNAIGEAFACVGLQVDAEA

SEQ ID NO: 189 - protein, 97 aa, synthetic construct
  REGION 1..97: note = Obscurin O.18
SEAPRFLTRPLAFVVSEGKDATLSSQIVGDPPPEVTWEKDQQPITAGARFRLAQDGDVYRLEILDLQLSDSGQYVSRARNAIGEAFACVGLQVDAEG

SEQ ID NO: 190 - protein, 97 aa, synthetic construct
  REGION 1..97: note = Obscurin O.19
SGAPRFLTRPLAFVVSVGKLAMLSSQIVGNPTPQVSWEKDQQPVAAGARFRLLQDGDLYRLKILDLALGDSGQYVSRARNAIGEAFACVGLQVDAEA

SEQ ID NO: 191 - protein, 97 aa, synthetic construct
  REGION 1..97: note = Obscurin O.20
SGAPRFLTRPLAFVVSVGKDATLSSQIVGNPTPQVSWEKDKQPVTAGARFRLAQDGDLYRLKILDLQLSDSGQYVSRARNAIGEAFACLGLQVDAEA

SEQ ID NO: 192 - protein, 97 aa, synthetic construct
  REGION 1..97: note = Obscurin O.21
SGAPRFLTRPLAFVVSVGKDATLSSQIVGNPTPQVSWEKDQLPVTAGARFRLAQDGDLYRLKILDLTLSDSGQYVSRARNAIGEAFACVGLEVGAEA

SEQ ID NO: 193 - protein, 97 aa, synthetic construct
  REGION 1..97: note = Obscurin O.22
SGAPRFLTRPLSYVVSVGKDASLSSQIVGNPTPQVSWEKDQLPVTAGARFRLAQDGDLYRLKILDLQLSDSGQYVSRARNAIGEAFACVGLEVGAEA

SEQ ID NO: 194 - protein, 102 aa, synthetic construct
  REGION 1..102: note = Obscurin O.23
DQPQFSGAPRFLTRPLSYVVSVGKDASLSSQIVGNPTPQVSWEKDQLPVTAGARFRLAQDGDLYRLKILDLQLSDSGQYVSRARNAIGEAFACVGLEVGAEA

SEQ ID NO: 195 - protein, 97 aa, synthetic construct
  REGION 1..97: note = Obscurin O.24
SGAPRFLTRPKAFVVSVGKDATLSSQIVGNPFPQVSWEKDKQPVTAGVRFRLAQDGDLYRLKILDLQLSDSGQYVSRARNAIGEAFACLGLQVDAEA

SEQ ID NO: 196 - protein, 97 aa, synthetic construct
  REGION 1..97: note = Obscurin O.25
SGAPRFLTRPKASVVSVGKDATLSSQIVGNPFPQVSWEKDKQPVTAGVRFRLAQDGDLYRLKILDLQLSDSGQYVSRARNAHGEAFACLGLQVDAEA

SEQ ID NO: 197 - protein, 97 aa, synthetic construct
  REGION 1..97: note = Obscurin O.26
SGCPRFLTRPKASVVSVGKDATLSSQIVGNPFPQVSWEKDKQPVTAGVRFRLAQDGDLYRLKILDLQLSDSGQYVSRARNAHGEAFACLGLQVDAEA

SEQ ID NO: 198 - protein, 97 aa, synthetic construct
  REGION 1..97: note = Obscurin O.27
SGAPRFLTCPKASVVSVGKDATLSSQIVGNPFPQVSWEKDKQPVTAGVRFRLAQDGDLYRLKILDLQLSDSGQYVSRARNAHGEAFACLGLQVDAEA

SEQ ID NO: 199 - protein, 97 aa, synthetic construct
  REGION 1..97: note = Obscurin O.28
SGAPRFLTRPKASVVSVGKDATLSCQIVGNPFPQVSWEKDKQPVTAGVRFRLAQDGDLYRLKILDLQLSDSGQYVCRARNAHGEAFACLGLQVDAEA

SEQ ID NO: 200 - protein, 97 aa, synthetic construct
  REGION 1..97: note = Obscurin O.29
SGCPRFLTRPKASVVSVGKDATLSCQIVGNPFPQVSWEKDKQPVTAGVRFRLAQDGDLYRLKILDLQLSDSGQYVCRARNAHGEAFACLGLQVDAEA

SEQ ID NO: 201 - protein, 97 aa, synthetic construct
  REGION 1..97: note = Obscurin O.30
SGAPRFLTCPKASVVSVGKDATLSCQIVGNPFPQVSWEKDKQPVTAGVRFRLAQDGDLYRLKILDLQLSDSGQYVCRARNAHGEAFACLGLQVDAEA

SEQ ID NO: 202 - protein, 97 aa, synthetic construct
  REGION 1..97: note = Obscurin O.31
SGAPRFLTRPKASVVSVGKDATLSSQIVGNPFPQVSWEKDKQPVTAGVRFRLAQDGDLYRLKILDCQLSDSGQYVSRARNAHGEAFACLGLQCDAEA

SEQ ID NO: 203 - protein, 97 aa, synthetic construct
  REGION 1..97: note = Obscurin O.32
SGCPRFLTRPKASVVSVGKDATLSSQIVGNPFPQVSWEKDKQPVTAGVRFRLAQDGDLYRLKILDCQLSDSGQYVSRARNAHGEAFACLGLQCDAEA

SEQ ID NO: 204 - protein, 97 aa, synthetic construct
  REGION 1..97: note = Obscurin O.33
SGAPRFLTCPKASVVSVGKDATLSSQIVGNPFPQVSWEKDKQPVTAGVRFRLAQDGDLYRLKILDCQLSDSGQYVSRARNAHGEAFACLGLQCDAEA

SEQ ID NO: 205 - protein, 27 aa, synthetic construct
  REGION 1..27: note = N-
MYKDCIESTGDYFLLCDAEGPWGIILE

SEQ ID NO: 206 - protein, 10 aa, synthetic construct
  REGION 1..10: note = E2
NQQTAPVRYC

SEQ ID NO: 207 - protein, 23 aa, synthetic construct
  REGION 1..23: note = E3
TEYVTLIMTRGMMFVNMTPCQLN

SEQ ID NO: 208 - protein, 15 aa, synthetic construct
  REGION 1..15: note = E4
RGNPQFQRQPQWDDC

SEQ ID NO: 209 - protein, 5 aa, synthetic construct
  REGION 1..5: note = 209
ASTKG

SEQ ID NO: 210 - protein, 5 aa, synthetic construct
  REGION 1..5: note = 210
RTVAS

SEQ ID NO: 211 - protein, 355 aa, Homo sapiens
MDYTLDLSVTTVTDYYYPDIFSSPCDAELIQTNGKLLLAVFYCLLFVFSLLGNSLVILVLVVCKKLRSITDVYLLNLALSDLLFVFSFPFQTYYLLDQWVFGTVMCKVVSGFYYIGFYSSMFFITLMSVDRYLAVVHAVYALKVRTIRMGTTLCLAVWLTAIMATIPLLVFYQVASEDGVLQCYSFYNQQTLKWKIFTNFKMNILGLLIPFTIFMFCYIKILHQLKRCQNHNKTKAIRLVLIVVIASLLFWVPFNVVLFLTSLHSMHILDGCSISQQLTYATHVTEIISFTHCCVNPVIYAFVGEKFKKHLSEIFQKSCSQIFNYLGRQMPRESCEKSSSCQQHSSRSSSVDYIL

SEQ ID NO: 212 - protein, 445 aa, Homo sapiens
RAETGSKGQTAGELYQRWERYRRECQETLAAAEPPSGLACNGSFDMYVCWDYAAPNATARASCPWYLPWHHHVAAGFVLRQCGSDGQWGLWRDHTQCENPEKNEAFLDQRLILERLQVMYTVGYSLSLATLLLALLILSLFRRLHCTRNYIHINLFTSFMLRAAAILSRDRLLPRPGPYLGDQALALWNQALAACRTAQIVTQYCVGANYTWLLVEGVYLHSLLVLVGGSEEGHFRYYLLLGWGAPALFVIPWVIVRYLYENTQCWERNEVKAIWWIIRTPILMTILINFLIFIRILGILLSKLRTRQMRCRDYRLRLARSTLTLVPLLGVHEVVFAPVTEEQARGALRFAKLGFEIFLSSFQGFLVSVLYCFINKEVQSEIRRGWHHCRLRRSLGEEQRQLPERAFRALPSGSGPGEVPTSRGLSSGTLPGPGNEASRELESYC

SEQ ID NO: 213 - protein, 4 aa, synthetic construct
  REGION 1..4: note = 213
GGGS

SEQ ID NO: 214 - protein, 4 aa, synthetic construct
  REGION 1..4: note = 214
GGGG

SEQ ID NO: 215 - protein, 330 aa, synthetic construct
  DOMAIN 1..330: note = CH
ASTKGPSVFPLAPSSKSTSGGTAALGCLVKDYFPEPVTVSWNSGALTSGVHTFPAVLQSSGLYSLSSVVTVPSSSLGTQTYICNVNHKPSNTKVDKKVEPKSCDKTHTCPPCPAPEAAGGPSVFLFPPKPKDTLMISRTPEVTCVVVDVSHEDPEVKFNWYVDGVEVHNAKTKPREEQYNSTYRVVSVLTVLHQDWLNGKEYKCKVSNKALPAPIEKTISKAKGQPREPQVYTLPPSRDELTKNQVSLTCLVKGFYPSDIAVEWESNGQPENNYKTTPPVLDSDGSFFLYSKLTVDKSRWQQGNVFSCSVMHEALHNHYTQKSLSLSPGK

SEQ ID NO: 216 - protein, 448 aa, synthetic construct
  CHAIN 1..448: note = Chi-1-heavy chain
EVQLVESGGGLVKPGGSLKLSCAASGFTFSDYGMHWVRQAPEKGLEWVAFISSGSSTIYYADTVKGRFTISRDNAKNTLFLQMTSLRSEDTAIYYCTRLGPNWYFDVWGTGTTVTVSSASTKGPSVFPLAPSSKSTSGGTAALGCLVKDYFPEPVTVSWNSGALTSGVHTFPAVLQSSGLYSLSSVVTVPSSSLGTQTYICNVNHKPSNTKVDKKVEPKSCDKTHTCPPCPAPEAAGGPSVFLFPPKPKDTLMISRTPEVTCVVVDVSHEDPEVKFNWYVDGVEVHNAKTKPREEQYNSTYRVVSVLTVLHQDWLNGKEYKCKVSNKALPAPIEKTISKAKGQPREPQVYTLPPSRDELTKNQVSLTCLVKGFYPSDIAVEWESNGQPENNYKTTPPVLDSDGSFFLYSKLTVDKSRWQQGNVFSCSVMHEALHNHYTQKSLSLSPGK

SEQ ID NO: 217 - protein, 220 aa, synthetic construct
  CHAIN 1..220: note = Chi-1-light chain
DVVMTQTPLSLSVSLGDQASISCRSSQSLVHSNGNTYLYWYLQKPGQSPKLLIYKVSNRFSGVPDRFSGSGSGTDFTLKISRVEAEDLGVYFCSQSTHVPPLTFGAGTKLELKRTVAAPSVFIFPPSDEQLKSGTASVVCLLNNFYPREAKVQWKVDNALQSGNSQESVTEQDSKDSTYSLSSTLTLSKADYEKHKVYACEVTHQGLSSPVTKSFNRGEC

SEQ ID NO: 218 - protein, 444 aa, synthetic construct
  CHAIN 1..444: note = Chi-24 heavy chain
QVQLQQSDAELVKPGGSVKISCKVSGYTFTDYPIHWMKQRPEQGLEWMGYVFPRDGSTKYNEKFRVKATWTADKSSSTVYMQLNSLTSDDSAVYFCSRELTAYWGQGTTLRVSSASTKGPSVFPLAPSSKSTSGGTAALGCLVKDYFPEPVTVSWNSGALTSGVHTFPAVLQSSGLYSLSSVVTVPSSSLGTQTYICNVNHKPSNTKVDKKVEPKSCDKTHTCPPCPAPEAAGGPSVFLFPPKPKDTLMISRTPEVTCVVVDVSHEDPEVKFNWYVDGVEVHNAKTKPREEQYNSTYRVVSVLTVLHQDWLNGKEYKCKVSNKALPAPIEKTISKAKGQPREPQVYTLPPSRDELTKNQVSLTCLVKGFYPSDIAVEWESNGQPENNYKTTPPVLDSDGSFFLYSKLTVDKSRWQQGNVFSCSVMHEALHNHYTQKSLSLSPGK

SEQ ID NO: 219 - protein, 219 aa, synthetic construct
  CHAIN 1..219: note = Chi-24 light chain
DVVLTQTPLTLSVTIGQPASISCKSSQSLLHSNGKTYLNWLLQRPGQSPRRLIYLVSKLDSGVPDRFAGSGSGTDFTLKITRVEAEDLGVYYCAQGTHFPRTFGGGSKLEIRRTVAAPSVFIFPPSDEQLKSGTASVVCLLNNFYPREAKVQWKVDNALQSGNSQESVTEQDSKDSTYSLSSTLTLSKADYEKHKVYACEVTHQGLSSPVTKSFNRGEC

SEQ ID NO: 220 - protein, 448 aa, synthetic construct
  CHAIN 1..448: note = Chi-30 heavy chain
EVQLQQSGPELVKPGGSMKISCKASGYSFTGYTMNWVKQSHGKNPEWIGLINPYNGGTRNNQKFKDKATLTVDKSSSTAYMELLSLTSEDSAVYYCTRWGLRLAMDYWGQGTSVTVSSASTKGPSVFPLAPSSKSTSGGTAALGCLVKDYFPEPVTVSWNSGALTSGVHTFPAVLQSSGLYSLSSVVTVPSSSLGTQTYICNVNHKPSNTKVDKKVEPKSCDKTHTCPPCPAPEAAGGPSVFLFPPKPKDTLMISRTPEVTCVVVDVSHEDPEVKFNWYVDGVEVHNAKTKPREEQYNSTYRVVSVLTVLHQDWLNGKEYKCKVSNKALPAPIEKTISKAKGQPREPQVYTLPPSRDELTKNQVSLTCLVKGFYPSDIAVEWESNGQPENNYKTTPPVLDSDGSFFLYSKLTVDKSRWQQGNVFSCSVMHEALHNHYTQKSLSLSPGK

SEQ ID NO: 221 - protein, 214 aa, synthetic construct
  CHAIN 1..214: note = Chi-30 light chain
DIVMTQSQKFMSTSVGDRVSVTCKASQNVGSNVAWYQQKPGQSPKALIYSASYRYSGVPDRFTGSGSGTDFTLTISNVQSEDLAEYFCHQYNSYPPTFGAGTKLALKRTVAAPSVFIFPPSDEQLKSGTASVVCLLNNFYPREAKVQWKVDNALQSGNSQESVTEQDSKDSTYSLSSTLTLSKADYEKHKVYACEVTHQGLSSPVTKSFNRGEC

SEQ ID NO: 222 - protein, 451 aa, synthetic construct
  CHAIN 1..451: note = Chi-45 heavy chain
EVKLVESGGGLVQPGDFLSLSCAASGFTFTDYYLSWVRQPPGKALEWLAFIRNRAKGYTTEYSASVKGRFTISRDNSQSILYLQMNVLRAEDSATYYCARMGGKGWHFDVWGTGTTVTVSSASTKGPSVFPLAPSSKSTSGGTAALGCLVKDYFPEPVTVSWNSGALTSGVHTFPAVLQSSGLYSLSSVVTVPSSSLGTQTYICNVNHKPSNTKVDKKVEPKSCDKTHTCPPCPAPEAAGGPSVFLFPPKPKDTLMISRTPEVTCVVVDVSHEDPEVKFNWYVDGVEVHNAKTKPREEQYNSTYRVVSVLTVLHQDWLNGKEYKCKVSNKALPAPIEKTISKAKGQPREPQVYTLPPSRDELTKNQVSLTCLVKGFYPSDIAVEWESNGQPENNYKTTPPVLDSDGSFFLYSKLTVDKSRWQQGNVFSCSVMHEALHNHYTQKSLSLSPGK

SEQ ID NO: 223 - protein, 219 aa, synthetic construct
  CHAIN 1..219: note = Chi-45 light chain
DVLMTQSPLSLPVSLGDQASISCRSSQSIVHSNGNTYLEWYLQKPGQSPKLLIYKVSNRFSGVPDRFFGSGSGTDFTLKINRVEAEDLGVYYCFQGSHVPFTFGGGTKLEIKRTVAAPSVFIFPPSDEQLKSGTASVVCLLNNFYPREAKVQWKVDNALQSGNSQESVTEQDSKDSTYSLSSTLTLSKADYEKHKVYACEVTHQGLSSPVTKSFNRGEC

SEQ ID NO: 224 - protein, 700 aa, synthetic construct
  CHAIN 1..700: note = F11-17 line1
EVQLVESGGGLVKPGGSLKLSCAASGFTFSDYGMHWVRQAPEKGLEWVAFISSGSSTIYYADTVKGRFTISRDNAKNTLFLQMTSLRSEDTAIYYCTRLGPNWYFDVWGTGTTVTVSSASTKGPSVFPLAPSSKSTSGGTAALGCLVKDYFPEPVTVSWNSGALTSGVHTFPAVLQSSGLYSLSSVVTVPSSSLGTQTYICNVNHKPSNTKVDKKVEPKSCEVQLVESGGGLVQPGGSLKLSCAASGFTFNKYAMNWVRQAPGKGLEWVARIRSKYNNYATYYADSVKDRFTISRDDSKNTAYLQMNNLKTEDTAVYYCVRHGNFGNEYISYWAYWGQGTLVTVSSGGGGSGGGGSGGGGSQTVVTQEPSLTVSPGGTVTLTCGSSTGAVTSGNYPNWVQQKPGQAPRGLIGGTKFLAPGTPARFSGSLLGGKAALTLSGVQPEDEAEYYCVLWYSNRWVFGGGTKLTVLGGGDKTHTCPPCPAPEAAGGPSVFLFPPKPKDTLMISRTPEVTCVVVDVSHEDPEVKFNWYVDGVEVHNAKTKPREEQYNSTYRVVSVLTVLHQDWLNGKEYKCKVSNKALPAPIEKTISKAKGQPREPQVYTLPPSRDELTKNQVSLTCLVKGFYPSDIAVEWESNGQPENNYKTTPPVLDSDGSFFLYSKLTVDKSRWQQGNVFSCSVMHEALHNHYTQKSLSLSPGK

SEQ ID NO: 225 - protein, 696 aa, synthetic construct
  CHAIN 1..696: note = F11-18 line1
QVQLQQSDAELVKPGGSVKISCKVSGYTFTDYPIHWMKQRPEQGLEWMGYVFPRDGSTKYNEKFRVKATWTADKSSSTVYMQLNSLTSDDSAVYFCSRELTAYWGQGTTLRVSSASTKGPSVFPLAPSSKSTSGGTAALGCLVKDYFPEPVTVSWNSGALTSGVHTFPAVLQSSGLYSLSSVVTVPSSSLGTQTYICNVNHKPSNTKVDKKVEPKSCEVQLVESGGGLVQPGGSLKLSCAASGFTFNKYAMNWVRQAPGKGLEWVARIRSKYNNYATYYADSVKDRFTISRDDSKNTAYLQMNNLKTEDTAVYYCVRHGNFGNEYISYWAYWGQGTLVTVSSGGGGSGGGGSGGGGSQTVVTQEPSLTVSPGGTVTLTCGSSTGAVTSGNYPNWVQQKPGQAPRGLIGGTKFLAPGTPARFSGSLLGGKAALTLSGVQPEDEAEYYCVLWYSNRWVFGGGTKLTVLGGGDKTHTCPPCPAPEAAGGPSVFLFPPKPKDTLMISRTPEVTCVVVDVSHEDPEVKFNWYVDGVEVHNAKTKPREEQYNSTYRVVSVLTVLHQDWLNGKEYKCKVSNKALPAPIEKTISKAKGQPREPQVYTLPPSRDELTKNQVSLTCLVKGFYPSDIAVEWESNGQPENNYKTTPPVLDSDGSFFLYSKLTVDKSRWQQGNVFSCSVMHEALHNHYTQKSLSLSPGK

SEQ ID NO: 226 - protein, 700 aa, synthetic construct
  CHAIN 1..700: note = F11-19 line1
EVQLQQSGPELVKPGGSMKISCKASGYSFTGYTMNWVKQSHGKNPEWIGLINPYNGGTRNNQKFKDKATLTVDKSSSTAYMELLSLTSEDSAVYYCTRWGLRLAMDYWGQGTSVTVSSASTKGPSVFPLAPSSKSTSGGTAALGCLVKDYFPEPVTVSWNSGALTSGVHTFPAVLQSSGLYSLSSVVTVPSSSLGTQTYICNVNHKPSNTKVDKKVEPKSCEVQLVESGGGLVQPGGSLKLSCAASGFTFNKYAMNWVRQAPGKGLEWVARIRSKYNNYATYYADSVKDRFTISRDDSKNTAYLQMNNLKTEDTAVYYCVRHGNFGNEYISYWAYWGQGTLVTVSSGGGGSGGGGSGGGGSQTVVTQEPSLTVSPGGTVTLTCGSSTGAVTSGNYPNWVQQKPGQAPRGLIGGTKFLAPGTPARFSGSLLGGKAALTLSGVQPEDEAEYYCVLWYSNRWVFGGGTKLTVLGGGDKTHTCPPCPAPEAAGGPSVFLFPPKPKDTLMISRTPEVTCVVVDVSHEDPEVKFNWYVDGVEVHNAKTKPREEQYNSTYRVVSVLTVLHQDWLNGKEYKCKVSNKALPAPIEKTISKAKGQPREPQVYTLPPSRDELTKNQVSLTCLVKGFYPSDIAVEWESNGQPENNYKTTPPVLDSDGSFFLYSKLTVDKSRWQQGNVFSCSVMHEALHNHYTQKSLSLSPGK

SEQ ID NO: 227 - protein, 451 aa, synthetic construct
  CHAIN 1..451: note = F4-9-line3
EVKLVESGGGLVQPGDFLSLSCAASGFTFTDYYLSWVRQPPGKALEWLAFIRNRAKGYTTEYSASVKGRFTISRDNSQSILYLQMNVLRAEDSATYYCARMGGKGWHFDVWGTGTTVTVSSASTKGPSVFPLAPSSKSTSGGTAALGCLVKDYFPEPVTVSWNSGALTSGVHTFPAVLQSSGLYSLSSVVTVPSSSLGTQTYICNVNHKPSNTKVDKKVEPKSCDKTHTCPPCPAPEAAGGPSVFLFPPKPKDTLMISRTPEVTCVVVDVSHEDPEVKFNWYVDGVEVHNAKTKPREEQYNSTYRVVSVLTVLHQDWLNGKEYKCKVSNKALPAPIEKTISKAKGQPREPQVCTLPPSRDELTKNQVSLSCAVKGFYPSDIAVEWESNGQPENNYKTTPPVLDSDGSFFLVSKLTVDKSRWQQGNVFSCSVMHEALHNHYTQKSLSLSPGK